European Patent Application EP 4 684 808 A1, published January 28, 2026. Title: Plasmids, Transgenes, Vectors and Medical Uses Comprising ADAMTS13. Applicant: Evotec International GmbH. Application EP. The sequence listing filed with the application follows.

SEQUENCE LISTING (42 sequences)

SEQ ID NO: 1 - DNA, 3474 bp, synthetic construct
  source 1..3474: mol_type = other DNA
atgcaccagcgtcacccccgggcaagatgccctcccctctgtgtggccggaatccttgcctgtggctttctcctgggctgctggggaccctcccatttccagcagagttgtcttcaggctttggagccacaggccgtgtcttcttacttgagccctggtgctcccttaaaaggccgccctccttcccctggcttccagaggcagaggcagaggcagaggcgggctgcaggcggcatcctacacctggagctgctggtggccgtgggccccgatgtcttccaggctcaccaggaggacacagagcgctatgtgctcaccaacctcaacatcggggcagaactgcttcgggacccgtccctgggggctcagtttcgggtgcacctggtgaagatggtcattctgacagagcctgagggtgctccaaatatcacagccaacctcacctcgtccctgctgagcgtctgtgggtggagccagaccatcaaccctgaggacgacacagatcctggccatgctgacctggtcctctatatcactaggtttgacctggagttgcctgatggtaaccggcaggtgcggggcgtcacccagctgggcggtgcctgctccccaacctggagctgcctcattaccgaggacactggcttcgacctgggagtcaccattgcccatgagattgggcacagcttcggcctggagcacgacggagcgcccggcagcggctgcggccccagcggacacgtgatggcttcggacggagctgctcctagagctggcctcgcttggtccccctgcagcagacggcagctgctgagcctgctcagcgcaggacgggcgcgctgcgtgtgggacccgccgcggcctcaacccgggtccgcggggcacccgccggatgcgcagcctggcctctactacagcgccaacgagcagtgccgcgtggccttcggccccaaggctgtcgcctgcaccttcgccagggagcacctggatatgtgccaggccctctcctgccacacagacccgctggaccaaagcagctgcagccgcctcctcgttcctctcctggatgggacagaatgtggcgtggagaagtggtgctccaagggtcgctgccgctccctggtggagctgacccccatagcagcagtgcatgggcgctggtctagctggggtccccgaagtccttgctcccgctcctgcggaggaggtgtggtcaccaggaggcggcagtgcaacaaccccagacctgcctttggggggcgtgcatgtgttggtgctgacctccaggccgagatgtgcaacactcaggcctgcgagaagacccagctggagttcatgtcgcaacagtgcgccaggaccgacggccagccgctgcgctcctcccctggcggcgcctccttctaccactggggtgctgctgtaccacacagccaaggggatgctctgtgcagacacatgtgccgggccattggcgagagcttcatcatgaagcgtggagacagcttcctcgatgggacccggtgtatgccaagtggcccccgggaggacgggaccctgagcctgtgtgtgtcgggcagctgcaggacatttggctgtgatggtaggatggactcccagcaggtatgggacaggtgccaggtgtgtggtggggacaacagcacgtgcagcccacggaagggctctttcacagctggcagagcgagagaatatgtcacgtttctgacagttacccccaacctgaccagtgtctacattgccaaccacaggcctctcttcacacacttggcggtgaggatcggagggcgctatgtcgtggctgggaagatgagcatctcccctaacaccacctacccctccctcctggaggatggtcgtgtcgagtacagagtggccctcaccgaggaccggctgccccgcctggaggagatccgcatctggggacccctccaggaagatgctgacatccaggtttacaggcggtatggcgaggagtatggcaacctcacccgcccagacatcaccttcacctacttccagcctaagccacggcaggcctgggtgtgggccgctgtgcgtgggccctgctcggtgagctgtggggcagggctgcgctgggtaaactacagctgcctggaccaggccaggaaggagttggtggagactgtccagtgccaagggagccagcagccaccagcgtggccagaggcctgcgtgctcgaaccctgccctccctactggaaagtcatgtcccttggcccatgttcggccagctgtggccttggcactgctagacgctcggtggcctgtgtgcagctcgaccaaggccaggacgtggaggtggacgaggcggcctgtgcggcgctggtgcggcccgaggccagtgtcccctgtctcattgccgactgcacctaccgctggcatgttggcacctggatggagtgctctgtttcctgtggggatggcatccagcgccggcgtgacacctgcctcggaccccaggcccaggcgcctgtgccagctgatttctgccagcacttgcccaagccggtgactgtgcgtggctgctgggctgggccctgtgtgggacagggtacgcccagcctggtgccccacgaagaagccgctgctccaggacggaccacagccacccctgctggtgcctccctggagtggtcccaggcccggggcctgctcttctccccggctccccagcctcggcggctcctgcccgggccccaggaaaactcagtgcagtccagtgcctgtggcaggcagcaccttgagccaacaggaaccattgacatgcgaggcccagggcaggcagactgtgcagtggccattgggcggcccctcggggaggtggtgaccctccgcgtccttgagagttctctcaactgcagtgcgggggacatgttgctgctttggggccggctcacctggaggaagatgtgcaggaagctgttggacatgactttcagctccaagaccaacacgctggtggtgaggcagcgctgcgggcggccaggaggtggggtgctgctgcggtatgggagccagcttgctcctgaaaccttctacagagaatgtgacatgcagctctttgggccctggggtgaaatcgtgagcccctcgctgagtccagccacgagtaatgcagggggctgccggctcttcattaatgtggctccgcacgcacggattgccatccatgccctggccaccaacatgggcgctgggaccgagggagccaatgccagctacatcttgatccgggacacccacagcttgaggaccacagcgtttcatgggcagcaggtgctctactgggagtcagagagcagccaggctgagatggagttcagcgagggcttcctgaaggctcaggccagcctgcggggccagtattggaccctccaatcatgggtaccggagatgcaggaccctcagtcctggaagggaaaggaaggaacctga

SEQ ID NO: 2 - protein, 1157 aa, synthetic construct
MHQRHPRARCPPLCVAGILACGFLLGCWGPSHFQQSCLQALEPQAVSSYLSPGAPLKGRPPSPGFQRQRQRQRRAAGGILHLELLVAVGPDVFQAHQEDTERYVLTNLNIGAELLRDPSLGAQFRVHLVKMVILTEPEGAPNITANLTSSLLSVCGWSQTINPEDDTDPGHADLVLYITRFDLELPDGNRQVRGVTQLGGACSPTWSCLITEDTGFDLGVTIAHEIGHSFGLEHDGAPGSGCGPSGHVMASDGAAPRAGLAWSPCSRRQLLSLLSAGRARCVWDPPRPQPGSAGHPPDAQPGLYYSANEQCRVAFGPKAVACTFAREHLDMCQALSCHTDPLDQSSCSRLLVPLLDGTECGVEKWCSKGRCRSLVELTPIAAVHGRWSSWGPRSPCSRSCGGGVVTRRRQCNNPRPAFGGRACVGADLQAEMCNTQACEKTQLEFMSQQCARTDGQPLRSSPGGASFYHWGAAVPHSQGDALCRHMCRAIGESFIMKRGDSFLDGTRCMPSGPREDGTLSLCVSGSCRTFGCDGRMDSQQVWDRCQVCGGDNSTCSPRKGSFTAGRAREYVTFLTVTPNLTSVYIANHRPLFTHLAVRIGGRYVVAGKMSISPNTTYPSLLEDGRVEYRVALTEDRLPRLEEIRIWGPLQEDADIQVYRRYGEEYGNLTRPDITFTYFQPKPRQAWVWAAVRGPCSVSCGAGLRWVNYSCLDQARKELVETVQCQGSQQPPAWPEACVLEPCPPYWKVMSLGPCSASCGLGTARRSVACVQLDQGQDVEVDEAACAALVRPEASVPCLIADCTYRWHVGTWMECSVSCGDGIQRRRDTCLGPQAQAPVPADFCQHLPKPVTVRGCWAGPCVGQGTPSLVPHEEAAAPGRTTATPAGASLEWSQARGLLFSPAPQPRRLLPGPQENSVQSSACGRQHLEPTGTIDMRGPGQADCAVAIGRPLGEVVTLRVLESSLNCSAGDMLLLWGRLTWRKMCRKLLDMTFSSKTNTLVVRQRCGRPGGGVLLRYGSQLAPETFYRECDMQLFGPWGEIVSPSLSPATSNAGGCRLFINVAPHARIAIHALATNMGAGTEGANASYILIRDTHSLRTTAFHGQQVLYWESESSQAEMEFSEGFLKAQASLRGQYWTLQSWVPEMQDPQSWKGKEGT

SEQ ID NO: 3 - DNA, 3825 bp, synthetic construct
  source 1..3825: mol_type = other DNA
tgtttgctgcttgcaatgtttgcccattttagggtggacacaggacgctgtggtttctgagccagggggcgactcagatcccagccagtggacttagcccctgtttgctcctccgataactggggtgaccttggttaatattcaccagcagcctcccccgttgcccctctggatccactgcttaaatacggacgaggacagggccctgtctcctcagcttcaggcaccaccactgacctgggacagtgaatccctcgaggggcgcgccgccaccatgcaccagcgtcacccccgggcaagatgccctcccctctgtgtggccggaatccttgcctgtggctttctcctgggctgctggggaccctcccatttccagcagagttgtcttcaggctttggagccacaggccgtgtcttcttacttgagccctggtgctcccttaaaaggccgccctccttcccctggcttccagaggcagaggcagaggcagaggcgggctgcaggcggcatcctacacctggagctgctggtggccgtgggccccgatgtcttccaggctcaccaggaggacacagagcgctatgtgctcaccaacctcaacatcggggcagaactgcttcgggacccgtccctgggggctcagtttcgggtgcacctggtgaagatggtcattctgacagagcctgagggtgctccaaatatcacagccaacctcacctcgtccctgctgagcgtctgtgggtggagccagaccatcaaccctgaggacgacacagatcctggccatgctgacctggtcctctatatcactaggtttgacctggagttgcctgatggtaaccggcaggtgcggggcgtcacccagctgggcggtgcctgctccccaacctggagctgcctcattaccgaggacactggcttcgacctgggagtcaccattgcccatgagattgggcacagcttcggcctggagcacgacggagcgcccggcagcggctgcggccccagcggacacgtgatggcttcggacggagctgctcctagagctggcctcgcttggtccccctgcagcagacggcagctgctgagcctgctcagcgcaggacgggcgcgctgcgtgtgggacccgccgcggcctcaacccgggtccgcggggcacccgccggatgcgcagcctggcctctactacagcgccaacgagcagtgccgcgtggccttcggccccaaggctgtcgcctgcaccttcgccagggagcacctggatatgtgccaggccctctcctgccacacagacccgctggaccaaagcagctgcagccgcctcctcgttcctctcctggatgggacagaatgtggcgtggagaagtggtgctccaagggtcgctgccgctccctggtggagctgacccccatagcagcagtgcatgggcgctggtctagctggggtccccgaagtccttgctcccgctcctgcggaggaggtgtggtcaccaggaggcggcagtgcaacaaccccagacctgcctttggggggcgtgcatgtgttggtgctgacctccaggccgagatgtgcaacactcaggcctgcgagaagacccagctggagttcatgtcgcaacagtgcgccaggaccgacggccagccgctgcgctcctcccctggcggcgcctccttctaccactggggtgctgctgtaccacacagccaaggggatgctctgtgcagacacatgtgccgggccattggcgagagcttcatcatgaagcgtggagacagcttcctcgatgggacccggtgtatgccaagtggcccccgggaggacgggaccctgagcctgtgtgtgtcgggcagctgcaggacatttggctgtgatggtaggatggactcccagcaggtatgggacaggtgccaggtgtgtggtggggacaacagcacgtgcagcccacggaagggctctttcacagctggcagagcgagagaatatgtcacgtttctgacagttacccccaacctgaccagtgtctacattgccaaccacaggcctctcttcacacacttggcggtgaggatcggagggcgctatgtcgtggctgggaagatgagcatctcccctaacaccacctacccctccctcctggaggatggtcgtgtcgagtacagagtggccctcaccgaggaccggctgccccgcctggaggagatccgcatctggggacccctccaggaagatgctgacatccaggtttacaggcggtatggcgaggagtatggcaacctcacccgcccagacatcaccttcacctacttccagcctaagccacggcaggcctgggtgtgggccgctgtgcgtgggccctgctcggtgagctgtggggcagggctgcgctgggtaaactacagctgcctggaccaggccaggaaggagttggtggagactgtccagtgccaagggagccagcagccaccagcgtggccagaggcctgcgtgctcgaaccctgccctccctactggaaagtcatgtcccttggcccatgttcggccagctgtggccttggcactgctagacgctcggtggcctgtgtgcagctcgaccaaggccaggacgtggaggtggacgaggcggcctgtgcggcgctggtgcggcccgaggccagtgtcccctgtctcattgccgactgcacctaccgctggcatgttggcacctggatggagtgctctgtttcctgtggggatggcatccagcgccggcgtgacacctgcctcggaccccaggcccaggcgcctgtgccagctgatttctgccagcacttgcccaagccggtgactgtgcgtggctgctgggctgggccctgtgtgggacagggtacgcccagcctggtgccccacgaagaagccgctgctccaggacggaccacagccacccctgctggtgcctccctggagtggtcccaggcccggggcctgctcttctccccggctccccagcctcggcggctcctgcccgggccccaggaaaactcagtgcagtccagtgcctgtggcaggcagcaccttgagccaacaggaaccattgacatgcgaggcccagggcaggcagactgtgcagtggccattgggcggcccctcggggaggtggtgaccctccgcgtccttgagagttctctcaactgcagtgcgggggacatgttgctgctttggggccggctcacctggaggaagatgtgcaggaagctgttggacatgactttcagctccaagaccaacacgctggtggtgaggcagcgctgcgggcggccaggaggtggggtgctgctgcggtatgggagccagcttgctcctgaaaccttctacagagaatgtgacatgcagctctttgggccctggggtgaaatcgtgagcccctcgctgagtccagccacgagtaatgcagggggctgccggctcttcattaatgtggctccgcacgcacggattgccatccatgccctggccaccaacatgggcgctgggaccgagggagccaatgccagctacatcttgatccgggacacccacagcttgaggaccacagcgtttcatgggcagcaggtgctctactgggagtcagagagcagccaggctgagatggagttcagcgagggcttcctgaaggctcaggccagcctgcggggccagtattggaccctccaatcatgggtaccggagatgcaggaccctcagtcctggaagggaaaggaaggaacctgataagcggccgcaatcaaagcttgagctcaataaaagatctttattttcattagatctgtgtgttggttttttgtgtg

SEQ ID NO: 4 - DNA, 4133 bp, synthetic construct
  source 1..4133: mol_type = other DNA
cctgcaggcagctgcgcgctcgctcgctcactgaggccgcccgggcgtcgggcgacctttggtcgcccggcctcagtgagcgagcgagcgcgcagagagggagtggccaactccatcactaggggttcctgcggccgcacgcgtgtgtttgctgcttgcaatgtttgcccattttagggtggacacaggacgctgtggtttctgagccagggggcgactcagatcccagccagtggacttagcccctgtttgctcctccgataactggggtgaccttggttaatattcaccagcagcctcccccgttgcccctctggatccactgcttaaatacggacgaggacagggccctgtctcctcagcttcaggcaccaccactgacctgggacagtgaatccctcgaggggcgcgccgccaccatgcaccagcgtcacccccgggcaagatgccctcccctctgtgtggccggaatccttgcctgtggctttctcctgggctgctggggaccctcccatttccagcagagttgtcttcaggctttggagccacaggccgtgtcttcttacttgagccctggtgctcccttaaaaggccgccctccttcccctggcttccagaggcagaggcagaggcagaggcgggctgcaggcggcatcctacacctggagctgctggtggccgtgggccccgatgtcttccaggctcaccaggaggacacagagcgctatgtgctcaccaacctcaacatcggggcagaactgcttcgggacccgtccctgggggctcagtttcgggtgcacctggtgaagatggtcattctgacagagcctgagggtgctccaaatatcacagccaacctcacctcgtccctgctgagcgtctgtgggtggagccagaccatcaaccctgaggacgacacagatcctggccatgctgacctggtcctctatatcactaggtttgacctggagttgcctgatggtaaccggcaggtgcggggcgtcacccagctgggcggtgcctgctccccaacctggagctgcctcattaccgaggacactggcttcgacctgggagtcaccattgcccatgagattgggcacagcttcggcctggagcacgacggagcgcccggcagcggctgcggccccagcggacacgtgatggcttcggacggagctgctcctagagctggcctcgcttggtccccctgcagcagacggcagctgctgagcctgctcagcgcaggacgggcgcgctgcgtgtgggacccgccgcggcctcaacccgggtccgcggggcacccgccggatgcgcagcctggcctctactacagcgccaacgagcagtgccgcgtggccttcggccccaaggctgtcgcctgcaccttcgccagggagcacctggatatgtgccaggccctctcctgccacacagacccgctggaccaaagcagctgcagccgcctcctcgttcctctcctggatgggacagaatgtggcgtggagaagtggtgctccaagggtcgctgccgctccctggtggagctgacccccatagcagcagtgcatgggcgctggtctagctggggtccccgaagtccttgctcccgctcctgcggaggaggtgtggtcaccaggaggcggcagtgcaacaaccccagacctgcctttggggggcgtgcatgtgttggtgctgacctccaggccgagatgtgcaacactcaggcctgcgagaagacccagctggagttcatgtcgcaacagtgcgccaggaccgacggccagccgctgcgctcctcccctggcggcgcctccttctaccactggggtgctgctgtaccacacagccaaggggatgctctgtgcagacacatgtgccgggccattggcgagagcttcatcatgaagcgtggagacagcttcctcgatgggacccggtgtatgccaagtggcccccgggaggacgggaccctgagcctgtgtgtgtcgggcagctgcaggacatttggctgtgatggtaggatggactcccagcaggtatgggacaggtgccaggtgtgtggtggggacaacagcacgtgcagcccacggaagggctctttcacagctggcagagcgagagaatatgtcacgtttctgacagttacccccaacctgaccagtgtctacattgccaaccacaggcctctcttcacacacttggcggtgaggatcggagggcgctatgtcgtggctgggaagatgagcatctcccctaacaccacctacccctccctcctggaggatggtcgtgtcgagtacagagtggccctcaccgaggaccggctgccccgcctggaggagatccgcatctggggacccctccaggaagatgctgacatccaggtttacaggcggtatggcgaggagtatggcaacctcacccgcccagacatcaccttcacctacttccagcctaagccacggcaggcctgggtgtgggccgctgtgcgtgggccctgctcggtgagctgtggggcagggctgcgctgggtaaactacagctgcctggaccaggccaggaaggagttggtggagactgtccagtgccaagggagccagcagccaccagcgtggccagaggcctgcgtgctcgaaccctgccctccctactggaaagtcatgtcccttggcccatgttcggccagctgtggccttggcactgctagacgctcggtggcctgtgtgcagctcgaccaaggccaggacgtggaggtggacgaggcggcctgtgcggcgctggtgcggcccgaggccagtgtcccctgtctcattgccgactgcacctaccgctggcatgttggcacctggatggagtgctctgtttcctgtggggatggcatccagcgccggcgtgacacctgcctcggaccccaggcccaggcgcctgtgccagctgatttctgccagcacttgcccaagccggtgactgtgcgtggctgctgggctgggccctgtgtgggacagggtacgcccagcctggtgccccacgaagaagccgctgctccaggacggaccacagccacccctgctggtgcctccctggagtggtcccaggcccggggcctgctcttctccccggctccccagcctcggcggctcctgcccgggccccaggaaaactcagtgcagtccagtgcctgtggcaggcagcaccttgagccaacaggaaccattgacatgcgaggcccagggcaggcagactgtgcagtggccattgggcggcccctcggggaggtggtgaccctccgcgtccttgagagttctctcaactgcagtgcgggggacatgttgctgctttggggccggctcacctggaggaagatgtgcaggaagctgttggacatgactttcagctccaagaccaacacgctggtggtgaggcagcgctgcgggcggccaggaggtggggtgctgctgcggtatgggagccagcttgctcctgaaaccttctacagagaatgtgacatgcagctctttgggccctggggtgaaatcgtgagcccctcgctgagtccagccacgagtaatgcagggggctgccggctcttcattaatgtggctccgcacgcacggattgccatccatgccctggccaccaacatgggcgctgggaccgagggagccaatgccagctacatcttgatccgggacacccacagcttgaggaccacagcgtttcatgggcagcaggtgctctactgggagtcagagagcagccaggctgagatggagttcagcgagggcttcctgaaggctcaggccagcctgcggggccagtattggaccctccaatcatgggtaccggagatgcaggaccctcagtcctggaagggaaaggaaggaacctgataagcggccgcaatcaaagcttgagctcaataaaagatctttattttcattagatctgtgtgttggttttttgtgtggtcgaccggaccgagcggccgcaggaacccctagtgatggagttggccactccctctctgcgcgctcgctcgctcactgaggccgggcgaccaaaggtcgcccgacgcccgggctttgcccgggcggcctcagtgagcgagcgagcgcgcagctgcctgcagg

SEQ ID NO: 5 - DNA, 6730 bp, synthetic construct
  source 1..6730: mol_type = other DNA
cctgcaggcagctgcgcgctcgctcgctcactgaggccgcccgggcgtcgggcgacctttggtcgcccggcctcagtgagcgagcgagcgcgcagagagggagtggccaactccatcactaggggttcctgcggccgcacgcgtgtgtttgctgcttgcaatgtttgcccattttagggtggacacaggacgctgtggtttctgagccagggggcgactcagatcccagccagtggacttagcccctgtttgctcctccgataactggggtgaccttggttaatattcaccagcagcctcccccgttgcccctctggatccactgcttaaatacggacgaggacagggccctgtctcctcagcttcaggcaccaccactgacctgggacagtgaatccctcgaggggcgcgccgccaccatgcaccagcgtcacccccgggcaagatgccctcccctctgtgtggccggaatccttgcctgtggctttctcctgggctgctggggaccctcccatttccagcagagttgtcttcaggctttggagccacaggccgtgtcttcttacttgagccctggtgctcccttaaaaggccgccctccttcccctggcttccagaggcagaggcagaggcagaggcgggctgcaggcggcatcctacacctggagctgctggtggccgtgggccccgatgtcttccaggctcaccaggaggacacagagcgctatgtgctcaccaacctcaacatcggggcagaactgcttcgggacccgtccctgggggctcagtttcgggtgcacctggtgaagatggtcattctgacagagcctgagggtgctccaaatatcacagccaacctcacctcgtccctgctgagcgtctgtgggtggagccagaccatcaaccctgaggacgacacagatcctggccatgctgacctggtcctctatatcactaggtttgacctggagttgcctgatggtaaccggcaggtgcggggcgtcacccagctgggcggtgcctgctccccaacctggagctgcctcattaccgaggacactggcttcgacctgggagtcaccattgcccatgagattgggcacagcttcggcctggagcacgacggagcgcccggcagcggctgcggccccagcggacacgtgatggcttcggacggagctgctcctagagctggcctcgcttggtccccctgcagcagacggcagctgctgagcctgctcagcgcaggacgggcgcgctgcgtgtgggacccgccgcggcctcaacccgggtccgcggggcacccgccggatgcgcagcctggcctctactacagcgccaacgagcagtgccgcgtggccttcggccccaaggctgtcgcctgcaccttcgccagggagcacctggatatgtgccaggccctctcctgccacacagacccgctggaccaaagcagctgcagccgcctcctcgttcctctcctggatgggacagaatgtggcgtggagaagtggtgctccaagggtcgctgccgctccctggtggagctgacccccatagcagcagtgcatgggcgctggtctagctggggtccccgaagtccttgctcccgctcctgcggaggaggtgtggtcaccaggaggcggcagtgcaacaaccccagacctgcctttggggggcgtgcatgtgttggtgctgacctccaggccgagatgtgcaacactcaggcctgcgagaagacccagctggagttcatgtcgcaacagtgcgccaggaccgacggccagccgctgcgctcctcccctggcggcgcctccttctaccactggggtgctgctgtaccacacagccaaggggatgctctgtgcagacacatgtgccgggccattggcgagagcttcatcatgaagcgtggagacagcttcctcgatgggacccggtgtatgccaagtggcccccgggaggacgggaccctgagcctgtgtgtgtcgggcagctgcaggacatttggctgtgatggtaggatggactcccagcaggtatgggacaggtgccaggtgtgtggtggggacaacagcacgtgcagcccacggaagggctctttcacagctggcagagcgagagaatatgtcacgtttctgacagttacccccaacctgaccagtgtctacattgccaaccacaggcctctcttcacacacttggcggtgaggatcggagggcgctatgtcgtggctgggaagatgagcatctcccctaacaccacctacccctccctcctggaggatggtcgtgtcgagtacagagtggccctcaccgaggaccggctgccccgcctggaggagatccgcatctggggacccctccaggaagatgctgacatccaggtttacaggcggtatggcgaggagtatggcaacctcacccgcccagacatcaccttcacctacttccagcctaagccacggcaggcctgggtgtgggccgctgtgcgtgggccctgctcggtgagctgtggggcagggctgcgctgggtaaactacagctgcctggaccaggccaggaaggagttggtggagactgtccagtgccaagggagccagcagccaccagcgtggccagaggcctgcgtgctcgaaccctgccctccctactggaaagtcatgtcccttggcccatgttcggccagctgtggccttggcactgctagacgctcggtggcctgtgtgcagctcgaccaaggccaggacgtggaggtggacgaggcggcctgtgcggcgctggtgcggcccgaggccagtgtcccctgtctcattgccgactgcacctaccgctggcatgttggcacctggatggagtgctctgtttcctgtggggatggcatccagcgccggcgtgacacctgcctcggaccccaggcccaggcgcctgtgccagctgatttctgccagcacttgcccaagccggtgactgtgcgtggctgctgggctgggccctgtgtgggacagggtacgcccagcctggtgccccacgaagaagccgctgctccaggacggaccacagccacccctgctggtgcctccctggagtggtcccaggcccggggcctgctcttctccccggctccccagcctcggcggctcctgcccgggccccaggaaaactcagtgcagtccagtgcctgtggcaggcagcaccttgagccaacaggaaccattgacatgcgaggcccagggcaggcagactgtgcagtggccattgggcggcccctcggggaggtggtgaccctccgcgtccttgagagttctctcaactgcagtgcgggggacatgttgctgctttggggccggctcacctggaggaagatgtgcaggaagctgttggacatgactttcagctccaagaccaacacgctggtggtgaggcagcgctgcgggcggccaggaggtggggtgctgctgcggtatgggagccagcttgctcctgaaaccttctacagagaatgtgacatgcagctctttgggccctggggtgaaatcgtgagcccctcgctgagtccagccacgagtaatgcagggggctgccggctcttcattaatgtggctccgcacgcacggattgccatccatgccctggccaccaacatgggcgctgggaccgagggagccaatgccagctacatcttgatccgggacacccacagcttgaggaccacagcgtttcatgggcagcaggtgctctactgggagtcagagagcagccaggctgagatggagttcagcgagggcttcctgaaggctcaggccagcctgcggggccagtattggaccctccaatcatgggtaccggagatgcaggaccctcagtcctggaagggaaaggaaggaacctgataagcggccgcaatcaaagcttgagctcaataaaagatctttattttcattagatctgtgtgttggttttttgtgtggtcgaccggaccgagcggccgcaggaacccctagtgatggagttggccactccctctctgcgcgctcgctcgctcactgaggccgggcgaccaaaggtcgcccgacgcccgggctttgcccgggcggcctcagtgagcgagcgagcgcgcagctgcctgcaggggcgcctgatgcggtattttctccttacgcatctgtgcggtatttcacaccgcatacgtcaaagcaaccatagtacgcgccctgtagcggcgcattaagcgcggcgggtgtggtggttacgcgcagcgtgaccgctacacttgccagcgccctagcgcccgctcctttcgctttcttcccttcctttctcgccacgttcgccggctttccccgtcaagctctaaatcgggggctccctttagggttccgatttagtgctttacggcacctcgaccccaaaaaacttgatttgggtgatggttcacgtagtgggccatcgccctgatagacggtttttcgccctttgacgttggagtccacgttctttaatagtggactcttgttccaaactggaacaacactcaaccctatctcgggctattcttttgatttataagggattttgccgatttcggcctattggttaaaaaatgagctgatttaacaaaaatttaacgcgaattttaacaaaatattaacgtttacaattttatggtgcactctcagtacaatctgctctgatgccgcatagttaagccagccccgacacccgccaacacccgctgacgcgccctgacgggcttgtctgctcccggcatccgcttacagacaagctgtgaccgtctccgggagctgcatgtgtcagaggttttcaccgtcatcaccgaaacgcgcgagacgaaagggcctcgtgatacgcctatttttataggttaatgtcatgataataatggtttcttagacgtcaggtggcacttttcggggaaatgtgcgcggaacccctatttgtttatttttctaaatacattcaaatatgtatccgctcatgagacaataaccctgataaatgcttcaataatattgaaaaaggaagagtatgagtattcaacatttccgtgtcgcccttattcccttttttgcggcattttgccttcctgtttttgctcacccagaaacgctggtgaaagtaaaagatgctgaagatcagttgggtgcacgagtgggttacatcgaactggatctcaacagcggtaagatccttgagagttttcgccccgaagaacgttttccaatgatgagcacttttaaagttctgctatgtggcgcggtattatcccgtattgacgccgggcaagagcaactcggtcgccgcatacactattctcagaatgacttggttgagtactcaccagtcacagaaaagcatcttacggatggcatgacagtaagagaattatgcagtgctgccataaccatgagtgataacactgcggccaacttacttctgacaacgatcggaggaccgaaggagctaaccgcttttttgcacaacatgggggatcatgtaactcgccttgatcgttgggaaccggagctgaatgaagccataccaaacgacgagcgtgacaccacgatgcctgtagcaatggcaacaacgttgcgcaaactattaactggcgaactacttactctagcttcccggcaacaattaatagactggatggaggcggataaagttgcaggaccacttctgcgctcggcccttccggctggctggtttattgctgataaatctggagccggtgagcgtgggtctcgcggtatcattgcagcactggggccagatggtaagccctcccgtatcgtagttatctacacgacggggagtcaggcaactatggatgaacgaaatagacagatcgctgagataggtgcctcactgattaagcattggtaactgtcagaccaagtttactcatatatactttagattgatttaaaacttcatttttaatttaaaaggatctaggtgaagatcctttttgataatctcatgaccaaaatcccttaacgtgagttttcgttccactgagcgtcagaccccgtagaaaagatcaaaggatcttcttgagatcctttttttctgcgcgtaatctgctgcttgcaaacaaaaaaaccaccgctaccagcggtggtttgtttgccggatcaagagctaccaactctttttccgaaggtaactggcttcagcagagcgcagataccaaatactgtccttctagtgtagccgtagttaggccaccacttcaagaactctgtagcaccgcctacatacctcgctctgctaatcctgttaccagtggctgctgccagtggcgataagtcgtgtcttaccgggttggactcaagacgatagttaccggataaggcgcagcggtcgggctgaacggggggttcgtgcacacagcccagcttggagcgaacgacctacaccgaactgagatacctacagcgtgagctatgagaaagcgccacgcttcccgaagggagaaaggcggacaggtatccggtaagcggcagggtcggaacaggagagcgcacgagggagcttccagggggaaacgcctggtatctttatagtcctgtcgggtttcgccacctctgacttgagcgtcgatttttgtgatgctcgtcaggggggcggagcctatggaaaaacgccagcaacgcggcctttttacggttcctggccttttgctggccttttgctcacatgt

SEQ ID NO: 6 - DNA, 262 bp, synthetic construct
  source 1..262: mol_type = other DNA
gtgagcgggcgggacggcccttctccttcgggctgtaattagcgcttggtttaatgacggcttgtttcttttctgtggctgcgtgaaagccttgaggggctccgggagggccctttgtgcggggggagcggctcggggctgtccgcggggggacggctgccttcgggggggacggggcagggcggggttcggcttctggcgtgtgaccggcggctctagagcctctgctaaccatgttcatgccttcttctttttcctacag

SEQ ID NO: 7 - DNA, 248 bp, synthetic construct
  source 1..248: mol_type = other DNA
aatcaacctctggattacaaaatttgtgaaagattgactggtattcttaactatgttgctccttttacgctatgtggatacgctgctttaatgcctttgtatcatgctattgcttcccgtatggctttcattttctcctccttgtataaatcctggttagttcttgccacggcggaactcatcgccgcctgccttgcccgctgctggacaggggctcggctgttgggcactgacaattccgtggtgtt

SEQ ID NO: 8 - DNA, 139 bp, synthetic construct
  source 1..139: mol_type = other DNA
tgcaggcagctgcgcgctcgctcgctcactgaggccgcccgggcaaagcccgggcgtcgggcgacctttggtcgcccggcctcagtgagcgagcgagcgcgcagagagggagtggccaactccatcactaggggttcct

SEQ ID NO: 9 - DNA, 139 bp, synthetic construct
  source 1..139: mol_type = other DNA
aggaacccctagtgatggagttggccactccctctctgcgcgctcgctcgctcactgaggccgggcgaccaaaggtcgcccgacgcccgggctttgcccgggcggcctcagtgagcgagcgagcgcgcagctgcctgca

SEQ ID NO: 10 - DNA, 4284 bp, synthetic construct
  source 1..4284: mol_type = other DNA
atgcaccagcgtcacccccgggcaagatgccctcccctctgtgtggccggaatccttgcctgtggctttctcctgggctgctggggaccctcccatttccagcagagttgtcttcaggctttggagccacaggccgtgtcttcttacttgagccctggtgctcccttaaaaggccgccctccttcccctggcttccagaggcagaggcagaggcagaggcgggctgcaggcggcatcctacacctggagctgctggtggccgtgggccccgatgtcttccaggctcaccaggaggacacagagcgctatgtgctcaccaacctcaacatcggggcagaactgcttcgggacccgtccctgggggctcagtttcgggtgcacctggtgaagatggtcattctgacagagcctgagggtgctccaaatatcacagccaacctcacctcgtccctgctgagcgtctgtgggtggagccagaccatcaaccctgaggacgacacagatcctggccatgctgacctggtcctctatatcactaggtttgacctggagttgcctgatggtaaccggcaggtgcggggcgtcacccagctgggcggtgcctgctccccaacctggagctgcctcattaccgaggacactggcttcgacctgggagtcaccattgcccatgagattgggcacagcttcggcctggagcacgacggagcgcccggcagcggctgcggccccagcggacacgtgatggcttcggacggagctgctcctagagctggcctcgcttggtccccctgcagcagacggcagctgctgagcctgctcagcgcaggacgggcgcgctgcgtgtgggacccgccgcggcctcaacccgggtccgcggggcacccgccggatgcgcagcctggcctctactacagcgccaacgagcagtgccgcgtggccttcggccccaaggctgtcgcctgcaccttcgccagggagcacctggatatgtgccaggccctctcctgccacacagacccgctggaccaaagcagctgcagccgcctcctcgttcctctcctggatgggacagaatgtggcgtggagaagtggtgctccaagggtcgctgccgctccctggtggagctgacccccatagcagcagtgcatgggcgctggtctagctggggtccccgaagtccttgctcccgctcctgcggaggaggtgtggtcaccaggaggcggcagtgcaacaaccccagacctgcctttggggggcgtgcatgtgttggtgctgacctccaggccgagatgtgcaacactcaggcctgcgagaagacccagctggagttcatgtcgcaacagtgcgccaggaccgacggccagccgctgcgctcctcccctggcggcgcctccttctaccactggggtgctgctgtaccacacagccaaggggatgctctgtgcagacacatgtgccgggccattggcgagagcttcatcatgaagcgtggagacagcttcctcgatgggacccggtgtatgccaagtggcccccgggaggacgggaccctgagcctgtgtgtgtcgggcagctgcaggacatttggctgtgatggtaggatggactcccagcaggtatgggacaggtgccaggtgtgtggtggggacaacagcacgtgcagcccacggaagggctctttcacagctggcagagcgagagaatatgtcacgtttctgacagttacccccaacctgaccagtgtctacattgccaaccacaggcctctcttcacacacttggcggtgaggatcggagggcgctatgtcgtggctgggaagatgagcatctcccctaacaccacctacccctccctcctggaggatggtcgtgtcgagtacagagtggccctcaccgaggaccggctgccccgcctggaggagatccgcatctggggacccctccaggaagatgctgacatccaggtttacaggcggtatggcgaggagtatggcaacctcacccgcccagacatcaccttcacctacttccagcctaagccacggcaggcctgggtgtgggccgctgtgcgtgggccctgctcggtgagctgtggggcagggctgcgctgggtaaactacagctgcctggaccaggccaggaaggagttggtggagactgtccagtgccaagggagccagcagccaccagcgtggccagaggcctgcgtgctcgaaccctgccctccctactgggcggtgggagacttcggcccatgcagcgcctcctgtgggggtggcctgcgggagcggccagtgcgctgcgtggaggcccagggcagcctcctgaagacattgcccccagcccggtgcagagcaggggcccagcagccagctgtggcgctggaaacctgcaacccccagccctgccctgccaggtgggaggtgtcagagcccagctcatgcacatcagctggtggagcaggcctggccttggagaacgagacctgtgtgccaggggcagatggcctggaggctccagtgactgaggggcctggctccgtagatgagaagctgcctgcccctgagccctgtgtcgggatgtcatgtcctccaggctggggccatctggatgccacctctgcaggggagaaggctccctccccttggggcagcatcaggacgggggctcaagctgcacacgtgtggacccctgcggcagggtcgtgctccgtctcctgcgggcgaggtctgatggagctgcgtttcctgtgcatggactctgccctcagggtgcctgtccaggaagagctgtgtggcctggcaagcaagcctgggagccggcgggaggtctgccaggctgtcccgtgccctgctcggtggcagtacaagctggcggcctgcagcgtgagctgtgggagaggggtcgtgcggagaatcctgtattgtgcccgggctcatggggaggacgatggtgaggagatcctgttggacacccagtgccaggggctgcctcgcccggaaccccaggaggcctgcagcctggagccctgcccacctaggtggaaagtcatgtcccttggcccatgttcggccagctgtggccttggcactgctagacgctcggtggcctgtgtgcagctcgaccaaggccaggacgtggaggtggacgaggcggcctgtgcggcgctggtgcggcccgaggccagtgtcccctgtctcattgccgactgcacctaccgctggcatgttggcacctggatggagtgctctgtttcctgtggggatggcatccagcgccggcgtgacacctgcctcggaccccaggcccaggcgcctgtgccagctgatttctgccagcacttgcccaagccggtgactgtgcgtggctgctgggctgggccctgtgtgggacagggtacgcccagcctggtgccccacgaagaagccgctgctccaggacggaccacagccacccctgctggtgcctccctggagtggtcccaggcccggggcctgctcttctccccggctccccagcctcggcggctcctgcccgggccccaggaaaactcagtgcagtccagtgcctgtggcaggcagcaccttgagccaacaggaaccattgacatgcgaggcccagggcaggcagactgtgcagtggccattgggcggcccctcggggaggtggtgaccctccgcgtccttgagagttctctcaactgcagtgcgggggacatgttgctgctttggggccggctcacctggaggaagatgtgcaggaagctgttggacatgactttcagctccaagaccaacacgctggtggtgaggcagcgctgcgggcggccaggaggtggggtgctgctgcggtatgggagccagcttgctcctgaaaccttctacagagaatgtgacatgcagctctttgggccctggggtgaaatcgtgagcccctcgctgagtccagccacgagtaatgcagggggctgccggctcttcattaatgtggctccgcacgcacggattgccatccatgccctggccaccaacatgggcgctgggaccgagggagccaatgccagctacatcttgatccgggacacccacagcttgaggaccacagcgtttcatgggcagcaggtgctctactgggagtcagagagcagccaggctgagatggagttcagcgagggcttcctgaaggctcaggccagcctgcggggccagtattggaccctccaatcatgggtaccggagatgcaggaccctcagtcctggaagggaaaggaaggaacctga

SEQ ID NO: 11 - DNA, 2061 bp, synthetic construct
  source 1..2061: mol_type = other DNA
atgcaccagcgtcacccccgggcaagatgccctcccctctgtgtggccggaatccttgcctgtggctttctcctgggctgctggggaccctcccatttccagcagagttgtcttcaggctttggagccacaggccgtgtcttcttacttgagccctggtgctcccttaaaaggccgccctccttcccctggcttccagaggcagaggcagaggcagaggcgggctgcaggcggcatcctacacctggagctgctggtggccgtgggccccgatgtcttccaggctcaccaggaggacacagagcgctatgtgctcaccaacctcaacatcggggcagaactgcttcgggacccgtccctgggggctcagtttcgggtgcacctggtgaagatggtcattctgacagagcctgagggtgctccaaatatcacagccaacctcacctcgtccctgctgagcgtctgtgggtggagccagaccatcaaccctgaggacgacacagatcctggccatgctgacctggtcctctatatcactaggtttgacctggagttgcctgatggtaaccggcaggtgcggggcgtcacccagctgggcggtgcctgctccccaacctggagctgcctcattaccgaggacactggcttcgacctgggagtcaccattgcccatgagattgggcacagcttcggcctggagcacgacggagcgcccggcagcggctgcggccccagcggacacgtgatggcttcggacggagctgctcctagagctggcctcgcttggtccccctgcagcagacggcagctgctgagcctgctcagcgcaggacgggcgcgctgcgtgtgggacccgccgcggcctcaacccgggtccgcggggcacccgccggatgcgcagcctggcctctactacagcgccaacgagcagtgccgcgtggccttcggccccaaggctgtcgcctgcaccttcgccagggagcacctggatatgtgccaggccctctcctgccacacagacccgctggaccaaagcagctgcagccgcctcctcgttcctctcctggatgggacagaatgtggcgtggagaagtggtgctccaagggtcgctgccgctccctggtggagctgacccccatagcagcagtgcatgggcgctggtctagctggggtccccgaagtccttgctcccgctcctgcggaggaggtgtggtcaccaggaggcggcagtgcaacaaccccagacctgcctttggggggcgtgcatgtgttggtgctgacctccaggccgagatgtgcaacactcaggcctgcgagaagacccagctggagttcatgtcgcaacagtgcgccaggaccgacggccagccgctgcgctcctcccctggcggcgcctccttctaccactggggtgctgctgtaccacacagccaaggggatgctctgtgcagacacatgtgccgggccattggcgagagcttcatcatgaagcgtggagacagcttcctcgatgggacccggtgtatgccaagtggcccccgggaggacgggaccctgagcctgtgtgtgtcgggcagctgcaggacatttggctgtgatggtaggatggactcccagcaggtatgggacaggtgccaggtgtgtggtggggacaacagcacgtgcagcccacggaagggctctttcacagctggcagagcgagagaatatgtcacgtttctgacagttacccccaacctgaccagtgtctacattgccaaccacaggcctctcttcacacacttggcggtgaggatcggagggcgctatgtcgtggctgggaagatgagcatctcccctaacaccacctacccctccctcctggaggatggtcgtgtcgagtacagagtggccctcaccgaggaccggctgccccgcctggaggagatccgcatctggggacccctccaggaagatgctgacatccaggtttacaggcggtatggcgaggagtatggcaacctcacccgcccagacatcaccttcacctacttccagcctaagccacggcaggcctgataa

SEQ ID NO: 12 - DNA, 6344 bp, synthetic construct
  source 1..6344: mol_type = other DNA
cctgcaggcagctgcgcgctcgctcgctcactgaggccgcccgggcgtcgggcgacctttggtcgcccggcctcagtgagcgagcgagcgcgcagagagggagtggccaactccatcactaggggttcctgcggccgcacgcgtggagctagttattaatagtaatcaattacggggtcattagttcatagcccatatatggagttccgcgttacataacttacggtaaatggcccgcctggctgaccgcccaacgacccccgcccattgacgtcaataatgacgtatgttcccatagtaacgtcaatagggactttccattgacgtcaatgggtggagtatttacggtaaactgcccacttggcagtacatcaagtgtatcatatgccaagtacgccccctattgacgtcaatgacggtaaatggcccgcctggcattatgcccagtacatgaccttatgggactttcctacttggcagtacatctacgtattagtcatcgctattaccatggtgatgcggttttggcagtacatcaatgggcgtggatagcggtttgactcacggggatttccaagtctccaccccattgacgtcaatgggagtttgttttgcaccaaaatcaacgggactttccaaaatgtcgtaacaactccgccccattgacgcaaatgggcggtaggcgtgtacggtgggaggtctatataagcagagctcgtttagtgaaccgtcagatcgcctggagacgccatccacgctgttttgacctccatagaagacaccgggaccgatccagcctccgcggattcgaatcccggccgggaacggtgcattggaacgcggattccccgtgccaagagtgacgtaagtaccgcctatagagtctataggcccacaaaaaatgctttcttcttttaatatacttttttgtttatcttatttctaatactttccctaatctctttctttcagggcaataatgatacaatgtatcatgcctctttgcaccattctaaagaataacagtgataatttctgggttaaggcaatagcaatatttctgcatataaatatttctgcatataaattgtaactgatgtaagaggtttcatattgctaatagcagctacaatccagctaccattctgcttttattttatggttgggataaggctggattattctgagtccaagctaggcccttttgctaatcatgttcatacctcttatcttcctcccacagctcctgggcaacgtgctggtctgtgtgctggcccatcactttggcaaagaattgggattcgaacatcgattgaattcgaattggatcctcgaggggcgcgccgccaccatgcaccagcgtcacccccgggcaagatgccctcccctctgtgtggccggaatccttgcctgtggctttctcctgggctgctggggaccctcccatttccagcagagttgtcttcaggctttggagccacaggccgtgtcttcttacttgagccctggtgctcccttaaaaggccgccctccttcccctggcttccagaggcagaggcagaggcagaggcgggctgcaggcggcatcctacacctggagctgctggtggccgtgggccccgatgtcttccaggctcaccaggaggacacagagcgctatgtgctcaccaacctcaacatcggggcagaactgcttcgggacccgtccctgggggctcagtttcgggtgcacctggtgaagatggtcattctgacagagcctgagggtgctccaaatatcacagccaacctcacctcgtccctgctgagcgtctgtgggtggagccagaccatcaaccctgaggacgacacagatcctggccatgctgacctggtcctctatatcactaggtttgacctggagttgcctgatggtaaccggcaggtgcggggcgtcacccagctgggcggtgcctgctccccaacctggagctgcctcattaccgaggacactggcttcgacctgggagtcaccattgcccatgagattgggcacagcttcggcctggagcacgacggagcgcccggcagcggctgcggccccagcggacacgtgatggcttcggacggagctgctcctagagctggcctcgcttggtccccctgcagcagacggcagctgctgagcctgctcagcgcaggacgggcgcgctgcgtgtgggacccgccgcggcctcaacccgggtccgcggggcacccgccggatgcgcagcctggcctctactacagcgccaacgagcagtgccgcgtggccttcggccccaaggctgtcgcctgcaccttcgccagggagcacctggatatgtgccaggccctctcctgccacacagacccgctggaccaaagcagctgcagccgcctcctcgttcctctcctggatgggacagaatgtggcgtggagaagtggtgctccaagggtcgctgccgctccctggtggagctgacccccatagcagcagtgcatgggcgctggtctagctggggtccccgaagtccttgctcccgctcctgcggaggaggtgtggtcaccaggaggcggcagtgcaacaaccccagacctgcctttggggggcgtgcatgtgttggtgctgacctccaggccgagatgtgcaacactcaggcctgcgagaagacccagctggagttcatgtcgcaacagtgcgccaggaccgacggccagccgctgcgctcctcccctggcggcgcctccttctaccactggggtgctgctgtaccacacagccaaggggatgctctgtgcagacacatgtgccgggccattggcgagagcttcatcatgaagcgtggagacagcttcctcgatgggacccggtgtatgccaagtggcccccgggaggacgggaccctgagcctgtgtgtgtcgggcagctgcaggacatttggctgtgatggtaggatggactcccagcaggtatgggacaggtgccaggtgtgtggtggggacaacagcacgtgcagcccacggaagggctctttcacagctggcagagcgagagaatatgtcacgtttctgacagttacccccaacctgaccagtgtctacattgccaaccacaggcctctcttcacacacttggcggtgaggatcggagggcgctatgtcgtggctgggaagatgagcatctcccctaacaccacctacccctccctcctggaggatggtcgtgtcgagtacagagtggccctcaccgaggaccggctgccccgcctggaggagatccgcatctggggacccctccaggaagatgctgacatccaggtttacaggcggtatggcgaggagtatggcaacctcacccgcccagacatcaccttcacctacttccagcctaagccacggcaggcctgggtgtgggccgctgtgcgtgggccctgctcggtgagctgtggggcagggctgcgctgggtaaactacagctgcctggaccaggccaggaaggagttggtggagactgtccagtgccaagggagccagcagccaccagcgtggccagaggcctgcgtgctcgaaccctgccctccctactgggcggtgggagacttcggcccatgcagcgcctcctgtgggggtggcctgcgggagcggccagtgcgctgcgtggaggcccagggcagcctcctgaagacattgcccccagcccggtgcagagcaggggcccagcagccagctgtggcgctggaaacctgcaacccccagccctgccctgccaggtgggaggtgtcagagcccagctcatgcacatcagctggtggagcaggcctggccttggagaacgagacctgtgtgccaggggcagatggcctggaggctccagtgactgaggggcctggctccgtagatgagaagctgcctgcccctgagccctgtgtcgggatgtcatgtcctccaggctggggccatctggatgccacctctgcaggggagaaggctccctccccttggggcagcatcaggacgggggctcaagctgcacacgtgtggacccctgcggcagggtcgtgctccgtctcctgcgggcgaggtctgatggagctgcgtttcctgtgcatggactctgccctcagggtgcctgtccaggaagagctgtgtggcctggcaagcaagcctgggagccggcgggaggtctgccaggctgtcccgtgccctgctcggtggcagtacaagctggcggcctgcagcgtgagctgtgggagaggggtcgtgcggagaatcctgtattgtgcccgggctcatggggaggacgatggtgaggagatcctgttggacacccagtgccaggggctgcctcgcccggaaccccaggaggcctgcagcctggagccctgcccacctaggtggaaagtcatgtcccttggcccatgttcggccagctgtggccttggcactgctagacgctcggtggcctgtgtgcagctcgaccaaggccaggacgtggaggtggacgaggcggcctgtgcggcgctggtgcggcccgaggccagtgtcccctgtctcattgccgactgcacctaccgctggcatgttggcacctggatggagtgctctgtttcctgtggggatggcatccagcgccggcgtgacacctgcctcggaccccaggcccaggcgcctgtgccagctgatttctgccagcacttgcccaagccggtgactgtgcgtggctgctgggctgggccctgtgtgggacagggtacgcccagcctggtgccccacgaagaagccgctgctccaggacggaccacagccacccctgctggtgcctccctggagtggtcccaggcccggggcctgctcttctccccggctccccagcctcggcggctcctgcccgggccccaggaaaactcagtgcagtccagtgcctgtggcaggcagcaccttgagccaacaggaaccattgacatgcgaggcccagggcaggcagactgtgcagtggccattgggcggcccctcggggaggtggtgaccctccgcgtccttgagagttctctcaactgcagtgcgggggacatgttgctgctttggggccggctcacctggaggaagatgtgcaggaagctgttggacatgactttcagctccaagaccaacacgctggtggtgaggcagcgctgcgggcggccaggaggtggggtgctgctgcggtatgggagccagcttgctcctgaaaccttctacagagaatgtgacatgcagctctttgggccctggggtgaaatcgtgagcccctcgctgagtccagccacgagtaatgcagggggctgccggctcttcattaatgtggctccgcacgcacggattgccatccatgccctggccaccaacatgggcgctgggaccgagggagccaatgccagctacatcttgatccgggacacccacagcttgaggaccacagcgtttcatgggcagcaggtgctctactgggagtcagagagcagccaggctgagatggagttcagcgagggcttcctgaaggctcaggccagcctgcggggccagtattggaccctccaatcatgggtaccggagatgcaggaccctcagtcctggaagggaaaggaaggaacctgataagcggccgcaatcaaagcttgcctcgagcagcgctgctcgagagatctacgggtggcatccctgtgacccctccccagtgcctctcctggccctggaagttgccactccagtgcccaccagccttgtcctaataaaattaagttgcatcattttgtctgactaggtgtccttctataatattatggggtggaggggggtggtatggagcaaggggcaagttgggaagacaacctgtagggcctgcggggtctattgggaaccaagctggagtgcagtggcacaatcttggctcactgcaatctccgcctcctgggttcaagcgattctcctgcctcagcctcccgagttgttgggattccaggcatgcatgaccaggctcagctaatttttgtttttttggtagagacggggtttcaccatattggccaggctggtctccaactcctaatctcaggtgatctacccaccttggcctcccaaattgctgggattacaggcgtgaaccactgctcccttccctgtccttctgattttgtaggtaaccacgtgcggaccgagcggccgcaggaacccctagtgatggagttggccactccctctctgcgcgctcgctcgctcactgaggccgggcgaccaaaggtcgcccgacgcccgggctttgcccgggcggcctcagtgagcgagcgagcgcgcagctgcctgcagg

SEQ ID NO: 13 - DNA, 6344 bp, synthetic construct
  source 1..6344: mol_type = other DNA
cctgcaggcagctgcgcgctcgctcgctcactgaggccgcccgggcgtcgggcgacctttggtcgcccggcctcagtgagcgagcgagcgcgcagagagggagtggccaactccatcactaggggttcctgcggccgcacgcgtggagctagttattaatagtaatcaattacggggtcattagttcatagcccatatatggagttccgcgttacataacttacggtaaatggcccgcctggctgaccgcccaacgacccccgcccattgacgtcaataatgacgtatgttcccatagtaacgtcaatagggactttccattgacgtcaatgggtggagtatttacggtaaactgcccacttggcagtacatcaagtgtatcatatgccaagtacgccccctattgacgtcaatgacggtaaatggcccgcctggcattatgcccagtacatgaccttatgggactttcctacttggcagtacatctacgtattagtcatcgctattaccatggtgatgcggttttggcagtacatcaatgggcgtggatagcggtttgactcacggggatttccaagtctccaccccattgacgtcaatgggagtttgttttgcaccaaaatcaacgggactttccaaaatgtcgtaacaactccgccccattgacgcaaatgggcggtaggcgtgtacggtgggaggtctatataagcagagctcgtttagtgaaccgtcagatcgcctggagacgccatccacgctgttttgacctccatagaagacaccgggaccgatccagcctccgcggattcgaatcccggccgggaacggtgcattggaacgcggattccccgtgccaagagtgacgtaagtaccgcctatagagtctataggcccacaaaaaatgctttcttcttttaatatacttttttgtttatcttatttctaatactttccctaatctctttctttcagggcaataatgatacaatgtatcatgcctctttgcaccattctaaagaataacagtgataatttctgggttaaggcaatagcaatatttctgcatataaatatttctgcatataaattgtaactgatgtaagaggtttcatattgctaatagcagctacaatccagctaccattctgcttttattttatggttgggataaggctggattattctgagtccaagctaggcccttttgctaatcatgttcatacctcttatcttcctcccacagctcctgggcaacgtgctggtctgtgtgctggcccatcactttggcaaagaattgggattcgaacatcgattgaattcgaattggatcctcgaggggcgcgccgccaccatgcaccagaggcatcctagagccagatgtcctcccctgtgtgtggctggcattctggcttgtggcttcctcctgggctgctggggtccttcccacttccagcagtcctgcctgcaagccctggaaccacaagctgtgtcctcctacctgtcccctggagcccccctcaagggaaggcccccctcccctggctttcagagacagaggcagagacaaagaagagcagctgggggcatcctgcacttggagctgctggttgctgtgggaccagatgtcttccaagcccaccaagaggacacagagagatatgttctgacaaacctgaacattggtgcagaactgctgagagatccctctctgggggcccagttcagagtccacctggtcaagatggtgatcctgactgagcctgaaggagcccccaacatcacagcaaacctcaccagctccctgctgtcagtgtgtggatggagccagaccatcaaccctgaggatgacacagatcctggccatgcagacctggtgctgtatatcaccagatttgacctggaactgcctgatgggaacagacaagtgaggggagtcacccagcttggaggtgcctgctcccctacctggtcatgtctgatcactgaagacactgggtttgatctgggtgtgactattgcccatgagattggccactcctttgggctggagcatgatggggctcctggaagtggctgtggcccatctggacatgtgatggcctcagatggggctgctccaagagctggcctggcatggtccccatgcagcagaagacagctcctgtctctgctgagtgctggcagagctaggtgtgtgtgggaccctcctaggcctcagcctgggtctgctgggcacccccctgatgcacagcctggcctgtactactctgccaatgagcagtgcagagtggcttttggccccaaagctgtggcctgcacatttgccagagagcacctggatatgtgccaagccctgtcctgccacacagaccccctggaccaatccagctgctctaggctgctggtgcctctcctggatggaacagaatgtggagtggaaaagtggtgctccaaaggaaggtgcagatccctggtggaactcacacccattgctgctgtccatggcagatggtcttcctggggccctaggagcccctgttccagatcctgtggaggaggggtggtgacaagaagaagacaatgcaacaacccccggcctgcctttggaggaagggcctgtgtgggagctgacctccaagcagagatgtgcaatacccaagcctgtgagaagacacagctggagttcatgtcacagcagtgtgccagaactgatggccagcccctgagaagctctcctgggggggcttccttctaccactggggggcagcagtcccccactctcaaggggatgccctctgccgccatatgtgtagagccattggagagagctttatcatgaagagaggtgacagcttccttgatggaaccagatgtatgcccagcgggcccagagaagatggcaccctgagcctctgtgtctctggctcctgcagaacctttggctgtgatggcagaatggactcccagcaagtctgggatagatgccaagtttgtgggggagacaacagcacctgtagccccagaaagggctctttcacagccggcagagccagagagtatgtcactttcctgactgtgaccccaaatctgacctctgtgtacattgccaaccacagaccactgtttacccatctggctgtgaggattgggggcagatatgtggtggctggaaaaatgtccatcagccctaacaccacctacccttcactgctggaggatggcagagtggagtacagagtggccctgacagaggacagactgcctagactggaggagatcagaatttggggccctctgcaagaagatgctgatatccaagtgtataggaggtatggggaggaatatggcaacctgaccagaccagacatcaccttcacctacttccagcccaagcccagacaagcctgggtttgggctgcagtgagaggcccctgctctgtgtcatgtggggctggcctgagatgggtgaactacagctgccttgaccaagccagaaaggagctggtggaaacagtccagtgccaaggctcccagcagccacctgcttggccagaagcctgtgtcctggagccttgtccaccctactgggcagtgggggactttggaccctgttctgcctcctgtggtggaggcctgagggaaagacctgtgagatgtgtggaggcacaaggaagcctgctgaaaaccctcccccctgccagatgtagagctggtgcccaacagcctgctgtggcactggagacatgtaatcctcagccctgccctgcaagatgggaagtcagtgagcccagttcctgcacctcagctggaggagctggactggccctggagaatgaaacttgtgttcctggagcagatggcctggaggccccagtcacagaaggccctggctctgttgatgagaaactgccagctcctgaaccttgtgtgggcatgtcttgccctcctggctggggacacctggatgccacttctgctggggagaaggctccctccccttggggcagcattaggactggagcccaagcagcccatgtgtggacacctgctgctggctcatgctcagtctcctgtggaaggggcctgatggagctgaggttcctgtgcatggattctgctctgagggtgcctgtgcaagaggagttgtgtggcttggcctccaagcctggcagtagaagggaggtctgccaagctgtgccctgcccagcccgctggcagtacaagctggctgcctgcagtgtcagctgtgggagaggagtggtgagaagaatcctgtactgtgcaagggctcatggagaggatgatggagaagaaatccttctggacacccagtgtcaaggcctgcccagacctgagccacaagaggcctgcagcctggaaccctgccccccaaggtggaaggtcatgagcctgggcccttgttcagcctcttgtggcctgggaactgccagaagatctgtggcttgtgtgcagctggatcaaggccaagatgtggaggtggatgaagcagcctgtgctgccctggtgaggccagaggccagtgtgccttgcctgattgcagattgtacctatagatggcatgttggcacatggatggagtgctctgtgagctgtggagatggtatccagaggagaagagacacctgcctgggacctcaagctcaagcccctgtccctgctgacttctgccagcatctgccaaagccagtgacagtgagggggtgctgggctgggccatgtgttggacaaggcaccccctccctggtgccccatgaagaggctgctgcacctggcagaaccactgctacccctgctggggcctccctggagtggagtcaagccagagggctgctcttcagcccagcaccccagcccagaagactgctgcctggcccccaagagaactctgtgcagtcttctgcatgtgggaggcagcaccttgagcccactggcaccattgacatgagagggcctgggcaagctgactgtgctgtggctattggcagacccctgggagaagtggtgaccctgagagtgctggaaagcagcctcaactgctctgctggagatatgctgctgctgtggggaagactgacctggagaaagatgtgtaggaagctcctggacatgaccttctccagcaagaccaacacactggtggtcagacagaggtgtggaagacctggaggaggagtgctgctgagatatggatctcagctggccccagagaccttctatagggagtgtgacatgcagctgtttggtccctggggggaaattgtgtctccatccctctccccagccacctccaatgctggaggctgcagactgttcatcaatgtggcccctcatgctagaattgccatccatgccctggccaccaacatgggagctggcactgagggggccaatgccagctacatcctcatcagagacacccacagcctgaggaccacagccttccatgggcagcaagtgctctactgggagtcagagtcctcccaagctgagatggaattttctgagggatttctgaaggcccaagcctccctgagaggccaatactggaccctgcagagctgggtgccagaaatgcaagacccacagtcatggaaaggcaaggaagggacctgataagcggccgcaatcaaagcttgcctcgagcagcgctgctcgagagatctacgggtggcatccctgtgacccctccccagtgcctctcctggccctggaagttgccactccagtgcccaccagccttgtcctaataaaattaagttgcatcattttgtctgactaggtgtccttctataatattatggggtggaggggggtggtatggagcaaggggcaagttgggaagacaacctgtagggcctgcggggtctattgggaaccaagctggagtgcagtggcacaatcttggctcactgcaatctccgcctcctgggttcaagcgattctcctgcctcagcctcccgagttgttgggattccaggcatgcatgaccaggctcagctaatttttgtttttttggtagagacggggtttcaccatattggccaggctggtctccaactcctaatctcaggtgatctacccaccttggcctcccaaattgctgggattacaggcgtgaaccactgctcccttccctgtccttctgattttgtaggtaaccacgtgcggaccgagcggccgcaggaacccctagtgatggagttggccactccctctctgcgcgctcgctcgctcactgaggccgggcgaccaaaggtcgcccgacgcccgggctttgcccgggcggcctcagtgagcgagcgagcgcgcagctgcctgcagg

SEQ ID NO: 14 - DNA, 6344 bp, synthetic construct
  source 1..6344: mol_type = other DNA
cctgcaggcagctgcgcgctcgctcgctcactgaggccgcccgggcgtcgggcgacctttggtcgcccggcctcagtgagcgagcgagcgcgcagagagggagtggccaactccatcactaggggttcctgcggccgcacgcgtggagctagttattaatagtaatcaattacggggtcattagttcatagcccatatatggagttccgcgttacataacttacggtaaatggcccgcctggctgaccgcccaacgacccccgcccattgacgtcaataatgacgtatgttcccatagtaacgtcaatagggactttccattgacgtcaatgggtggagtatttacggtaaactgcccacttggcagtacatcaagtgtatcatatgccaagtacgccccctattgacgtcaatgacggtaaatggcccgcctggcattatgcccagtacatgaccttatgggactttcctacttggcagtacatctacgtattagtcatcgctattaccatggtgatgcggttttggcagtacatcaatgggcgtggatagcggtttgactcacggggatttccaagtctccaccccattgacgtcaatgggagtttgttttgcaccaaaatcaacgggactttccaaaatgtcgtaacaactccgccccattgacgcaaatgggcggtaggcgtgtacggtgggaggtctatataagcagagctcgtttagtgaaccgtcagatcgcctggagacgccatccacgctgttttgacctccatagaagacaccgggaccgatccagcctccgcggattcgaatcccggccgggaacggtgcattggaacgcggattccccgtgccaagagtgacgtaagtaccgcctatagagtctataggcccacaaaaaatgctttcttcttttaatatacttttttgtttatcttatttctaatactttccctaatctctttctttcagggcaataatgatacaatgtatcatgcctctttgcaccattctaaagaataacagtgataatttctgggttaaggcaatagcaatatttctgcatataaatatttctgcatataaattgtaactgatgtaagaggtttcatattgctaatagcagctacaatccagctaccattctgcttttattttatggttgggataaggctggattattctgagtccaagctaggcccttttgctaatcatgttcatacctcttatcttcctcccacagctcctgggcaacgtgctggtctgtgtgctggcccatcactttggcaaagaattgggattcgaacatcgattgaattcgaattggatcctcgaggggcgcgccgccaccatgcaccagagacatcctagggccagatgtccccccctctgtgttgctggcatcctggcctgtggatttctgctgggctgctggggccctagccacttccagcagtcctgcctgcaagcccttgagccccaagctgtgtcctcctacctgtcccctggagcccccctaaagggcagacccccctcccctggctttcagagacagaggcaaaggcagaggagggcagctgggggcattctgcacctggagcttctggtggcagtgggccctgatgtcttccaagcccaccaagaagacactgagaggtatgttctgacaaacctcaacattggagcagagctgctgagagacccatctttgggggcccagttcagagtccacctggtcaaaatggtgatcctcacagagccagagggagccccaaatatcacagccaacctgacttcttctctgctgtctgtctgtggctggagccagaccatcaaccctgaagatgacacagaccctgggcatgctgacctagtgctctatatcaccagatttgacctggaactcccagatggaaacagacaagttagaggggttactcagcttgggggggcctgctcccccacctggagttgcctcatcactgaggacactggttttgatctgggggtcaccatagcccatgagattggccactcctttggtctggagcatgatggagcccctggctctggctgtggcccctctggccatgttatggcaagtgatggtgctgccccaagggctggcctggcttggtctccttgctcaaggaggcagctcctgtccctcctctctgctgggagggcaaggtgtgtgtgggaccccccaagacctcagcctggcagtgctggacaccctccagatgcacagcctggtctctactactctgccaatgaacagtgtagggtggcctttggccccaaggcagtagcctgcacatttgccagagagcacctggacatgtgccaagccctcagctgccacacagatccccttgaccagtccagctgctccagactcttggtgcccctgctggatgggacagaatgtggggtggaaaagtggtgcagcaaggggaggtgtaggagcctggttgaactgaccccaattgcagcagtgcatgggaggtggtcatcatggggtcctaggtccccctgcagtaggagttgtggggggggagtggtcacaaggaggaggcagtgcaataatcccagaccagcttttgggggtagggcctgtgtaggggcagacctccaagctgagatgtgtaatacccaagcctgtgagaaaacccaactggagttcatgagccagcagtgtgctaggactgatggccagcccctcagatccagccctggaggtgcctccttctaccactggggagcagcagtcccccactcacaaggggatgccctctgccgccatatgtgcagagccataggggaatcatttatcatgaagaggggggacagctttcttgatgggaccagatgtatgcctagtgggcctagggaagatgggacactgagcctatgtgtcagtgggtcctgcagaacctttggctgtgatggaagaatggactcccagcaagtgtgggataggtgccaagtgtgtggtggagacaactccacctgttccccaaggaaagggagcttcactgctggcagagctagggagtatgtcactttccttactgtcacccccaatctcacctctgtttacattgccaaccataggcccctgttcacccaccttgctgtaagaataggtggcagatatgtggtggctgggaagatgtccatctcccccaacaccacctaccccagcctgctggaggatggcagagtggagtatagggtggctcttacagaggacagactgccaaggttggaagaaataagaatctgggggccattgcaagaggatgctgacatccaagtgtacagaaggtatggggaggaatatggcaatctgacaagaccagacattacattcacatacttccagccaaagccaaggcaagcctgggtctgggcagcagtgagaggcccctgctcagtgtcctgtggtgctggcctaaggtgggtgaactacagctgcctggaccaagccagaaaagagctagttgagactgtacaatgccaaggcagccagcagccccctgcatggccagaagcctgtgtcctggaaccctgccccccctactgggctgttggtgactttggaccttgctcagccagctgtggaggggggcttagggagagaccagtgcggtgtgtggaggctcaaggctcactcctgaagaccctccccccagcaaggtgcagagctggggctcagcaacctgctgtggccttggagacctgcaacccccagccctgtcctgccagatgggaggtctctgaaccaagtagctgcacctcagctggtggggctgggctggcattggagaatgagacatgtgtgcctggtgcagatggcctggaggccccagtcacagaaggacctggaagtgttgatgagaagctgcctgcccctgagccctgtgtgggcatgtcttgcccccctggatggggccacctggatgccacaagtgctggggagaaggctccttcaccctggggaagcatcagaactggagcccaagcagcccatgtatggacccctgctgctgggtcatgctctgtgtcttgtggcagagggctgatggagctgaggttcctgtgcatggattctgctctgagggtgcctgtccaagaggagctgtgtgggttggcctctaagcctgggagcagaagggaagtctgccaagcagttccctgcccagccagatggcagtacaagctagcagcttgcagtgtcagctgtgggagaggggtggttaggaggattctttactgtgcaagggcccatggagaggatgatggggaagagatcctgttggacacccagtgccaagggctccctaggccagagccacaagaggcctgcagcctggagccttgccctcctagatggaaggtgatgtcactgggcccttgctctgcatcttgtggcctggggactgcaagaaggtctgtggcctgtgttcagttggatcaaggacaagatgtggaagtggatgaagctgcatgtgctgccctggtgaggccagaggcatcagtcccatgcctgattgctgactgcacttatagatggcatgtgggcacatggatggagtgcagtgtctcctgtggagatgggattcagagaaggagggacacctgccttggcccccaagcccaagcccctgtgccagcagacttctgccagcatctgcccaaacctgtgactgtgagggggtgttgggctggcccttgtgtggggcaaggaaccccttcccttgtccctcacgaggaggctgctgcccctgggaggaccacagcaactccagcgggtgccagccttgagtggtcccaagctaggggcctcctcttcagcccagccccccaacccagaaggctgttgcccggaccccaagagaactcagtgcagtcctcagcatgtgggaggcagcacttggaacccactggcaccattgatatgagaggtcctgggcaagctgactgtgcagttgccattgggaggccactgggagaggtggtgaccctgagagtgctagagtccagcctcaactgctcagctggagacatgctgttgctgtgggggaggctgacctggagaaagatgtgtaggaagctcttggacatgaccttctccagtaaaaccaacaccctggtggtcagacagaggtgtggaaggcctggtgggggtgtgctgctgaggtatggctcccagctagccccagaaaccttctatagggagtgtgacatgcagctgtttggaccatggggtgaaattgtgagcccctctctctccccagccacctccaatgctggaggctgtaggttgttcatcaatgtggccccccatgccagaattgccatccatgcactggccaccaacatgggggctggcacagagggggccaatgccagctacatcctcataagggacactcacagcctcagaaccactgccttccatggccagcaagtcctgtactgggaatctgagagcagccaagcagaaatggaattttcagagggcttcctcaaggcccaagccagtttgagggggcagtattggactctgcagtcctgggttcctgagatgcaagacccccagagctggaaaggcaaagaaggcacctgataagcggccgcaatcaaagcttgcctcgagcagcgctgctcgagagatctacgggtggcatccctgtgacccctccccagtgcctctcctggccctggaagttgccactccagtgcccaccagccttgtcctaataaaattaagttgcatcattttgtctgactaggtgtccttctataatattatggggtggaggggggtggtatggagcaaggggcaagttgggaagacaacctgtagggcctgcggggtctattgggaaccaagctggagtgcagtggcacaatcttggctcactgcaatctccgcctcctgggttcaagcgattctcctgcctcagcctcccgagttgttgggattccaggcatgcatgaccaggctcagctaatttttgtttttttggtagagacggggtttcaccatattggccaggctggtctccaactcctaatctcaggtgatctacccaccttggcctcccaaattgctgggattacaggcgtgaaccactgctcccttccctgtccttctgattttgtaggtaaccacgtgcggaccgagcggccgcaggaacccctagtgatggagttggccactccctctctgcgcgctcgctcgctcactgaggccgggcgaccaaaggtcgcccgacgcccgggctttgcccgggcggcctcagtgagcgagcgagcgcgcagctgcctgcagg

SEQ ID NO: 15 - DNA, 6344 bp, synthetic construct
  source 1..6344: mol_type = other DNA
cctgcaggcagctgcgcgctcgctcgctcactgaggccgcccgggcgtcgggcgacctttggtcgcccggcctcagtgagcgagcgagcgcgcagagagggagtggccaactccatcactaggggttcctgcggccgcacgcgtggagctagttattaatagtaatcaattacggggtcattagttcatagcccatatatggagttccgcgttacataacttacggtaaatggcccgcctggctgaccgcccaacgacccccgcccattgacgtcaataatgacgtatgttcccatagtaacgtcaatagggactttccattgacgtcaatgggtggagtatttacggtaaactgcccacttggcagtacatcaagtgtatcatatgccaagtacgccccctattgacgtcaatgacggtaaatggcccgcctggcattatgcccagtacatgaccttatgggactttcctacttggcagtacatctacgtattagtcatcgctattaccatggtgatgcggttttggcagtacatcaatgggcgtggatagcggtttgactcacggggatttccaagtctccaccccattgacgtcaatgggagtttgttttgcaccaaaatcaacgggactttccaaaatgtcgtaacaactccgccccattgacgcaaatgggcggtaggcgtgtacggtgggaggtctatataagcagagctcgtttagtgaaccgtcagatcgcctggagacgccatccacgctgttttgacctccatagaagacaccgggaccgatccagcctccgcggattcgaatcccggccgggaacggtgcattggaacgcggattccccgtgccaagagtgacgtaagtaccgcctatagagtctataggcccacaaaaaatgctttcttcttttaatatacttttttgtttatcttatttctaatactttccctaatctctttctttcagggcaataatgatacaatgtatcatgcctctttgcaccattctaaagaataacagtgataatttctgggttaaggcaatagcaatatttctgcatataaatatttctgcatataaattgtaactgatgtaagaggtttcatattgctaatagcagctacaatccagctaccattctgcttttattttatggttgggataaggctggattattctgagtccaagctaggcccttttgctaatcatgttcatacctcttatcttcctcccacagctcctgggcaacgtgctggtctgtgtgctggcccatcactttggcaaagaattgggattcgaacatcgattgaattcgaattggatcctcgaggggcgcgccgccaccatgcaccagagacatcctagagccagatgccctcccctgtgtgtggctggcatcctggcttgtggctttctgttgggctgctggggtccttcccacttccagcagagctgcctgcaagccctggagcctcaagcagtcagcagctacctgagtcctggagcccctctcaagggcagacccccctctcctgggtttcagaggcagaggcaaaggcagagaagggcagctggggggattctgcacctggagctgctggtggcagtgggccctgatgtcttccaagcccaccaagaggatactgagagatatgttctgaccaatctgaacattggggcagaactgctgagggacccatctctgggggcccagttcagagtgcatctggtgaagatggtgatcctgacagagccagagggagcccccaacatcactgcaaacctcacctcctctctgctgtcagtgtgtggatggagccagaccatcaaccctgaggatgacacagaccctggccatgcagatttggtgctctacatcaccagatttgatctggagcttccagatggaaacagacaagttagaggagtcacccagcttgggggagcctgctcccccacctggtcatgcctgatcacagaggacactggatttgacctgggtgtcacaattgcccatgaaataggccattcctttggactggagcatgatggggctcctggatctgggtgtggcccttctggacatgtgatggcctctgatggagcagcccccagagctggcttggcctggtctccatgctcaagaagacagctcctgtccctgctgtctgctggaagggccagatgtgtgtgggaccctcctaggccccagcccggatcagctggacacccccctgatgcccaacctgggctgtactactctgccaatgagcagtgtagagtggcctttggacctaaggcagtggcctgcacatttgccagagagcaccttgatatgtgtcaagctctctcctgccatactgatcccctggatcagagcagttgctccagactgctggtccccctcctggatggcacagaatgtggtgtggagaagtggtgctccaagggaaggtgcagatccctggtggaactcaccccaattgctgctgtccatggtaggtggagtagctgggggccaaggagcccatgtagcagatcctgtgggggtggagttgtgaccagaaggagacagtgcaacaacccaaggcctgcttttggtgggagggcctgtgtgggagctgacctccaagcagagatgtgcaatacccaagcctgtgagaagacccagttggagttcatgtctcagcagtgtgccagaacagatggccagcctctgagaagctctcctggtggggcttccttctaccactggggggctgctgtgccccacagccaaggtgatgccctctgtaggcatatgtgcagagccattggagagagctttatcatgaagagaggtgactctttcttggatgggaccagatgtatgcccagtggcccaagagaagatggcaccctgagcctgtgcgtgtctggcagctgtaggacttttggctgtgatggaagaatggactcccagcaagtgtgggataggtgtcaagtctgtggaggagacaacagcacatgcagccccagaaaaggcagcttcacagctggcagagcaagagagtatgtcaccttcctgactgtgacccccaatctgacctctgtgtacattgccaaccacagacccctgtttacacatctggctgtgagaattggtggcagatatgtggttgctggcaagatgagcatcagccctaacaccacctatccttcactgcttgaagatggaagggtggagtacagagttgccctgacagaagacagactgcctagattggaagagattaggatctggggaccattgcaagaggatgcagacatccaagtgtatagaaggtatggagaggaatatggcaacctgaccagacctgacattactttcacctacttccagcccaagcccagacaagcctgggtttgggcagcagtgaggggaccttgctctgtttcttgtggagctggcctgagatgggtgaactacagctgcctggatcaagcaagaaaggagctggttgagacagtccagtgccaaggctcacaacagcctccagcatggcccgaggcctgtgtccttgagccctgccccccctactgggccgtgggggattttggcccctgctctgcatcctgtggagggggcctgagagagaggccagtgagatgtgtggaagcacaaggctccctgctgaaaaccctccccccagctagatgcagagctggagcccagcagccagcagtggccctggaaacctgtaacccccagccatgccctgccagatgggaagtcagtgagcccagctcctgcacctcagctggaggtgctggcctggcactggagaatgaaacatgtgttcctggggctgatggtctggaggcacctgtgactgaggggcctggctctgtggatgaaaagctccctgcccctgaaccctgtgtagggatgtcatgtcctcctggctggggccacctggatgctaccagtgctggtgagaaagctccaagcccttggggctccatcagaactggtgcccaagcagcccatgtctggacacctgcagctggaagctgttctgtgagttgtgggagaggactcatggagctgaggttcctctgcatggattctgccctgcgggtgcctgtccaagaagaattgtgtgggctggcctccaaacctggctccagaagggaagtgtgccaagctgttccctgcccagccagatggcagtacaagctggctgcctgctctgtgtcatgtggaagaggggtggtcagaaggattctgtactgtgcaagggctcatggagaagatgatggggaggagatcttgctggacactcaatgccaaggcctcccaagacctgaaccacaagaagcctgcagcctggaaccttgtccacctagatggaaagtcatgtccctgggcccctgcagtgccagctgtggcctgggaacagccagaagatctgtggcttgtgtgcagcttgaccaaggacaagatgtggaggttgatgaggctgcatgtgctgccctggtgagaccagaggcttctgtcccttgtctgattgcagattgcacttacagatggcatgttggaacctggatggaatgcagtgtgagctgtggagatggtatccagagaagaagagatacctgccttggcccccaagctcaagccccagtgcctgctgacttctgccagcacctgcccaaaccagtgacagtgagagggtgctgggctggaccctgtgttgggcaagggacaccctccctggtgccccatgaggaggctgctgcccctggcagaaccacagcaacccctgctggggcctcattagagtggtcccaagctaggggcctgctgttctccccagcccctcagcctaggaggctgttgcctggccctcaagagaactcagtgcagtcttcagcctgtgggagacagcatctggagccaactggcaccattgatatgagaggccctggccaagctgactgtgctgtggctattggcagaccactgggagaggtggtgactctgagggtcctggaatcttccctcaactgctctgctggggacatgctgctgctgtggggcagactgacatggagaaaaatgtgtaggaaactgctggacatgaccttttccagcaagacaaacacactggtggtgagacaaagatgtggcagacctgggggaggagtgctgctcagatatgggtctcagctggcccctgagaccttctatagggagtgtgacatgcagctgtttgggccctggggagaaattgtgtccccatccctgtcccctgccacttccaatgctggaggctgtagactcttcatcaatgtggctcctcatgccagaatagccatccatgctctggccaccaacatgggagctggcactgaaggagccaatgcctcctacatcctcatcagagacacccactctctgaggaccactgccttccatgggcagcaagtgctgtactgggagtctgagtcctcccaagctgagatggagttttcagagggcttcctgaaggcccaagccagtctgagaggacagtattggaccctgcagtcctgggtgccagaaatgcaagacccccagtcatggaaggggaaggaaggcacctgataagcggccgcaatcaaagcttgcctcgagcagcgctgctcgagagatctacgggtggcatccctgtgacccctccccagtgcctctcctggccctggaagttgccactccagtgcccaccagccttgtcctaataaaattaagttgcatcattttgtctgactaggtgtccttctataatattatggggtggaggggggtggtatggagcaaggggcaagttgggaagacaacctgtagggcctgcggggtctattgggaaccaagctggagtgcagtggcacaatcttggctcactgcaatctccgcctcctgggttcaagcgattctcctgcctcagcctcccgagttgttgggattccaggcatgcatgaccaggctcagctaatttttgtttttttggtagagacggggtttcaccatattggccaggctggtctccaactcctaatctcaggtgatctacccaccttggcctcccaaattgctgggattacaggcgtgaaccactgctcccttccctgtccttctgattttgtaggtaaccacgtgcggaccgagcggccgcaggaacccctagtgatggagttggccactccctctctgcgcgctcgctcgctcactgaggccgggcgaccaaaggtcgcccgacgcccgggctttgcccgggcggcctcagtgagcgagcgagcgcgcagctgcctgcagg

SEQ ID NO: 16 - DNA, 6344 bp, synthetic construct
  source 1..6344: mol_type = other DNA
cctgcaggcagctgcgcgctcgctcgctcactgaggccgcccgggcgtcgggcgacctttggtcgcccggcctcagtgagcgagcgagcgcgcagagagggagtggccaactccatcactaggggttcctgcggccgcacgcgtggagctagttattaatagtaatcaattacggggtcattagttcatagcccatatatggagttccgcgttacataacttacggtaaatggcccgcctggctgaccgcccaacgacccccgcccattgacgtcaataatgacgtatgttcccatagtaacgtcaatagggactttccattgacgtcaatgggtggagtatttacggtaaactgcccacttggcagtacatcaagtgtatcatatgccaagtacgccccctattgacgtcaatgacggtaaatggcccgcctggcattatgcccagtacatgaccttatgggactttcctacttggcagtacatctacgtattagtcatcgctattaccatggtgatgcggttttggcagtacatcaatgggcgtggatagcggtttgactcacggggatttccaagtctccaccccattgacgtcaatgggagtttgttttgcaccaaaatcaacgggactttccaaaatgtcgtaacaactccgccccattgacgcaaatgggcggtaggcgtgtacggtgggaggtctatataagcagagctcgtttagtgaaccgtcagatcgcctggagacgccatccacgctgttttgacctccatagaagacaccgggaccgatccagcctccgcggattcgaatcccggccgggaacggtgcattggaacgcggattccccgtgccaagagtgacgtaagtaccgcctatagagtctataggcccacaaaaaatgctttcttcttttaatatacttttttgtttatcttatttctaatactttccctaatctctttctttcagggcaataatgatacaatgtatcatgcctctttgcaccattctaaagaataacagtgataatttctgggttaaggcaatagcaatatttctgcatataaatatttctgcatataaattgtaactgatgtaagaggtttcatattgctaatagcagctacaatccagctaccattctgcttttattttatggttgggataaggctggattattctgagtccaagctaggcccttttgctaatcatgttcatacctcttatcttcctcccacagctcctgggcaacgtgctggtctgtgtgctggcccatcactttggcaaagaattgggattcgaacatcgattgaattcgaattggatcctcgaggggcgcgccgccaccatgcaccagagacacccaagggctaggtgcccacctctgtgtgtggctggcatcttggcttgtggatttctccttggttgctggggacccagccacttccagcagtcctgcctgcaagccctggagcctcaagctgtctcctcctacctgagccctggtgcccccttgaaaggcagaccccctagccctgggttccaaagacagagacagaggcagagaagagctgctgggggaatcctgcacctggaactgctggtggctgtgggccctgatgtctttcaagcccaccaagaggacacagagagatatgttttgaccaacctgaatattggggcagagcttctaagggacccctctctgggagcccagtttagggtccacctggtcaagatggtgatccttacagaaccagaaggggctcccaacatcactgccaacctcaccagctccctcctctcagtatgtggctggtcacagaccatcaaccctgaggatgacactgaccctggacatgctgatctggttctctacatcacaaggtttgatttagagttaccagatggaaatagacaagtcagaggtgtaacccagcttgggggggcctgctcccccacctggagttgcctgatcacagaggacactggctttgacctgggtgtcacaatagctcatgaaattggtcactcatttggtctggaacatgatggggctcctggctctggctgtggcccttctggccatgtgatggcctctgatggagcagccccaagagctggattagcttggagcccatgcagcagaagacagctcctcagtctgctgtctgctgggagagcaaggtgtgtgtgggaccctcccagaccccaacctggatcagctgggcaccccccagatgctcagcctggcctgtactactctgcaaatgagcagtgcagagtggcttttggccctaaagcagtggcctgcacctttgctagagaacacttggacatgtgtcaagccctctcttgccacacagacccacttgaccagagttcctgctctaggctacttgtacccctcctagatgggactgagtgtggtgtggagaaatggtgctccaaagggagatgtaggtccctggtagagctgaccccaattgctgcagtacatggaaggtggtcttcctggggtcccagaagcccttgcagtagaagttgtgggggtggtgttgtgaccagaagaagacagtgcaacaaccccagaccagcctttggaggaagggcctgtgtgggggctgacctccaagctgagatgtgcaatacccaagcatgtgaaaagactcagttagagttcatgtcacagcagtgtgcaaggacagatggccagccactgaggtcatcccctggtggggcctccttctaccactggggtgctgcagtcccccacagccaaggggatgccctatgtaggcatatgtgcagagccattggagagagctttatcatgaagaggggtgactcctttctggatggtacaagatgcatgcccagtggccctagagaggatggcaccctgagtttgtgtgtctctggctcctgtaggacttttggctgtgatggaaggatggattctcagcaagtgtgggataggtgccaagtctgtggaggggacaattccacctgttcacctaggaagggcagcttcacagctggaagggccagagagtatgtgaccttccttactgtcacccccaatctcacaagtgtttatatagcaaaccaccgccccctcttcacacatctggctgtcagaataggagggagatatgtagttgctggcaaaatgtccatcagccccaacaccacctacccctcactgctggaagatggcagagttgaatatagggtggcactgactgaagataggttgccaaggttagaggagatcagaatttgggggccactccaagaagatgctgacatccaagtttacagaaggtatggtgaagaatatggaaaccttaccagacctgacattactttcacctatttccagcccaagccaaggcaagcctgggtttgggcagctgtgagggggccttgttctgtgagctgtggagctggcttgagatgggtgaactacagctgcttagaccaagccagaaaagaacttgtggagacagtccagtgtcaaggaagccagcagcccccagcatggccagaagcctgtgtgcttgaaccctgccccccctactgggcagtaggagactttggcccctgcagcgcctcatgtggggggggcttaagggagaggccagtgaggtgtgtagaagcccaaggatctctgctcaagacactgcctcctgccagatgtagagctggagcccagcagccagctgtggccttagagacctgcaatccacagccatgccctgcaaggtgggaagtttctgaaccctccagctgcacttcagctggaggagctggccttgccctggagaatgaaacttgtgtgcctggtgcagatggactggaggccccagtgacagaaggacctgggtctgttgatgaaaaacttcctgccccagagccatgtgttggcatgtcttgcccccctggatggggccacttagatgcaaccagtgctggagagaaggcccccagtccatggggcagtatcagaactggagcacaagctgcccatgtctggacaccagcagccggttcatgctcagtgtcctgtggaaggggcctgatggagttgagattcctctgtatggactcagcactaagggtcccagttcaagaggagctgtgtggcttggcatccaagcccggaagtagaagagaggtctgccaagcagtgccctgtccagccagatggcagtacaagctggctgcatgtagtgtcagctgtgggaggggggtggttagaagaattttgtactgtgccagagcccatggtgaggatgatggagaagagatactgctggacacccagtgccaaggtctcccaagaccggaacctcaagaggcctgctctttggagccctgccctcctaggtggaaagtcatgagcctggggccctgcagtgcctcttgtggcctgggcactgctaggaggtctgtggcctgtgtccaactggatcaaggccaagatgtggaggtggatgaggctgcttgtgctgccttagtgagaccagaggcatcagttccctgtctgattgcagactgtacctacagatggcatgttggaacctggatggagtgctcagtttcctgtggggatggtatccagagaaggagagacacatgcttaggccctcaagcacaagcccctgttcctgcagacttctgccagcacctccccaaacctgtgactgtgagaggctgctgggctggcccctgtgttgggcaaggcaccccttccctagtgccacatgaggaagctgctgcccctggcagaaccacagccactcctgctggagcttccctggagtggtcccaagcaaggggacttctgttctccccagcaccccagccaaggaggctcttgcctggcccacaagagaacagtgtgcagtcctctgcctgtggtagacagcatcttgagcccactggtactatagacatgaggggtcctgggcaagcagattgtgctgtagctattggcagacctcttggagaagtggtcactttgagggtgctggaatctagcctcaactgctctgctggtgacatgctgctgctgtggggaaggctcacatggagaaagatgtgtaggaaattgctggacatgaccttctcaagcaagaccaatactctggtggtgaggcagaggtgtggaagacctggtggaggggtactcctgaggtatggctcccagctagcccctgaaacattctatagggaatgtgatatgcagctgtttgggccctggggggagattgtcagtccttcactctcccctgctacctccaatgctggtgggtgcagactattcatcaatgtggctccccatgcaagaattgccatccatgccttggccaccaacatgggagctggaactgagggtgccaatgccagctacattctcatcagagatactcactctcttaggaccactgccttccatgggcagcaagtgctctactgggagagtgaaagctcacaagcagaaatggaattttctgagggcttcctgaaggctcaagcctccttgaggggccagtattggaccctgcagagctgggtccctgagatgcaagacccccagtcttggaagggaaaagaggggacctgataagcggccgcaatcaaagcttgcctcgagcagcgctgctcgagagatctacgggtggcatccctgtgacccctccccagtgcctctcctggccctggaagttgccactccagtgcccaccagccttgtcctaataaaattaagttgcatcattttgtctgactaggtgtccttctataatattatggggtggaggggggtggtatggagcaaggggcaagttgggaagacaacctgtagggcctgcggggtctattgggaaccaagctggagtgcagtggcacaatcttggctcactgcaatctccgcctcctgggttcaagcgattctcctgcctcagcctcccgagttgttgggattccaggcatgcatgaccaggctcagctaatttttgtttttttggtagagacggggtttcaccatattggccaggctggtctccaactcctaatctcaggtgatctacccaccttggcctcccaaattgctgggattacaggcgtgaaccactgctcccttccctgtccttctgattttgtaggtaaccacgtgcggaccgagcggccgcaggaacccctagtgatggagttggccactccctctctgcgcgctcgctcgctcactgaggccgggcgaccaaaggtcgcccgacgcccgggctttgcccgggcggcctcagtgagcgagcgagcgcgcagctgcctgcagg

SEQ ID NO: 17 - DNA, 6344 bp, synthetic construct
  source 1..6344: mol_type = other DNA
cctgcaggcagctgcgcgctcgctcgctcactgaggccgcccgggcgtcgggcgacctttggtcgcccggcctcagtgagcgagcgagcgcgcagagagggagtggccaactccatcactaggggttcctgcggccgcacgcgtggagctagttattaatagtaatcaattacggggtcattagttcatagcccatatatggagttccgcgttacataacttacggtaaatggcccgcctggctgaccgcccaacgacccccgcccattgacgtcaataatgacgtatgttcccatagtaacgtcaatagggactttccattgacgtcaatgggtggagtatttacggtaaactgcccacttggcagtacatcaagtgtatcatatgccaagtacgccccctattgacgtcaatgacggtaaatggcccgcctggcattatgcccagtacatgaccttatgggactttcctacttggcagtacatctacgtattagtcatcgctattaccatggtgatgcggttttggcagtacatcaatgggcgtggatagcggtttgactcacggggatttccaagtctccaccccattgacgtcaatgggagtttgttttgcaccaaaatcaacgggactttccaaaatgtcgtaacaactccgccccattgacgcaaatgggcggtaggcgtgtacggtgggaggtctatataagcagagctcgtttagtgaaccgtcagatcgcctggagacgccatccacgctgttttgacctccatagaagacaccgggaccgatccagcctccgcggattcgaatcccggccgggaacggtgcattggaacgcggattccccgtgccaagagtgacgtaagtaccgcctatagagtctataggcccacaaaaaatgctttcttcttttaatatacttttttgtttatcttatttctaatactttccctaatctctttctttcagggcaataatgatacaatgtatcatgcctctttgcaccattctaaagaataacagtgataatttctgggttaaggcaatagcaatatttctgcatataaatatttctgcatataaattgtaactgatgtaagaggtttcatattgctaatagcagctacaatccagctaccattctgcttttattttatggttgggataaggctggattattctgagtccaagctaggcccttttgctaatcatgttcatacctcttatcttcctcccacagctcctgggcaacgtgctggtctgtgtgctggcccatcactttggcaaagaattgggattcgaacatcgattgaattcgaattggatcctcgaggggcgcgccgccaccatgcaccagaggcacccaagggctaggtgcccccccctgtgtgtagctggcatcctggcctgtggcttcctcctggggtgctggggcccttcccacttccagcagagctgcctccaagccctggagccacaagcagtgagcagctacctgagccctggggcacccctgaaaggcagacccccctcccctgggtttcaaaggcagaggcagagacagaggagggcagctgggggcattctgcaccttgagctgctggtggctgtgggccctgatgtgttccaagcccaccaagaagacactgagagatatgtcctcaccaatctgaatataggagcagaattgctgagggacccatctctgggtgcccagtttagggtccacctagtgaagatggtgatcctcacagagcctgaaggggctcccaacatcactgccaatctcaccagcagcctcctgagtgtgtgtggctggtcccagaccatcaaccctgaggatgacactgaccctggccatgctgacctggtgctctatatcaccagatttgatttggaactgcctgatgggaataggcaagtcagaggagtcacccaactggggggggcctgctcacccacatggtcttgcctgatcacagaggacactggctttgacctgggggtgaccatagcccatgaaattggccactcctttggcttggagcatgatggggcacctggctctgggtgtggcccaagtggccatgtgatggcctctgatggggctgctcctagggctggactggcctggtcaccctgctctaggagacagctgctctccctcctctctgctggtagggccagatgtgtgtgggacccccccagaccccaacctggctcagctggccaccccccagatgcacagcctggcctctactactcagccaatgagcagtgcagagtggcatttggccccaaagctgtggcctgcacctttgctagggagcacttggacatgtgccaagccctctcctgccacacagaccccctagaccagtcctcctgctcaaggcttcttgtgcccctgctggatggcacagaatgtggggtggagaagtggtgctccaaggggaggtgtaggtccctggtggagctgacccccatagcagcagtccatgggaggtggagtagctggggacccagatccccctgcagtaggagctgtggtgggggggtggtcacccggaggaggcagtgcaacaacccaaggccagcctttggtggcagagcctgtgtaggggcagacctccaagcagagatgtgcaacactcaagcctgtgagaaaacccagctagagttcatgtcccagcagtgtgccagaacagatggccagcccctcagaagttcccctggaggggcctccttctaccactggggggctgcagtcccccacagtcaaggggatgcactctgtaggcatatgtgcagagccattggggagtcctttatcatgaagagaggggactccttcctggatgggactaggtgtatgccctctggccccagagaggatggcactctgtccctctgtgtgtctggctcctgcagaacttttggctgtgatgggaggatggatagccagcaagtgtgggacagatgccaagtctgtggaggagacaactccacctgcagccctaggaaggggagcttcacagctgggagggccagagaatatgtgactttcctgacagtgacccccaacctcacctctgtgtacattgccaaccataggcccctcttcacccacctggcagtcagaattggagggaggtatgtagtggctggcaagatgagcatcagccccaataccacctatcccagcctgctggaagatgggagggtggagtacagagtagccctgactgaagataggctgccaaggctggaggagatcagaatttgggggcccttacaagaggatgctgacatccaagtctataggaggtatggggaagagtatggcaacctgactaggccagacattaccttcacctacttccagcccaagccaaggcaagcctgggtctgggcagctgtcagaggcccttgcagtgtctcttgtggagctggcctgaggtgggtgaactactcctgccttgaccaagccagaaaggagctggtggagacagtccagtgccaaggcagccagcagcccccagcatggccagaggcctgtgtcttagagccctgccctccctactgggcagtgggggactttggcccctgctcagcctcatgtggggggggtctgagggagaggccagtgaggtgtgtggaagcccaagggtcactgctcaagaccctcccccctgccagatgtagggctggtgcccagcagccagctgttgccctggaaacctgcaatccccaaccctgccctgctaggtgggaggtctcagagccctccagctgcaccagtgctgggggggctggtctggcccttgagaatgaaacctgtgtgcctggggcagatggcctggaggcccctgtcactgagggcccggggtctgtggatgagaagctccctgccccagagccctgtgtgggcatgagctgcccccctggttggggccacctggatgccacttctgctggggaaaaagcacccagtccctgggggtccattaggactggggcacaagcagcccatgtctggaccccagctgccgggagttgctcagtcagctgtgggagggggctgatggagctgaggttcctctgcatggactctgcactgagggtcccagtccaagaggagctttgtgggcttgccagcaaacctggcagcagaagggaggtctgccaagctgtgccctgcccagccagatggcagtacaagctggctgcctgctctgttagctgtggcagaggggtggtgagaaggatcttgtactgtgctagagcacatggagaggatgatggtgaggaaatccttctggacacccagtgtcaaggcctccctaggcctgaaccccaagaggcctgcagcctggagccctgtcctcctaggtggaaggtcatgtcccttgggccctgctctgcctcctgtggactggggactgccagaagatcagttgcttgtgtgcagctggaccaaggccaagatgttgaggtagatgaagcagcctgtgctgccctggtgaggccagaagccagtgtcccctgtctgattgctgactgcacatataggtggcatgtggggacctggatggaatgctcagtgtcctgtggggatggtatccagaggaggagggacacatgcctgggcccccaagcccaagctcctgtgcctgcagacttctgccagcacctgcccaagcccgtcacagttaggggctgctgggctgggccctgtgttgggcaaggaacaccctccctggtcccccatgaggaggctgctgcccctgggaggaccacagccacccctgcgggggcctctctggagtggagccaagctagggggctcctgttctccccagccccccagcctagaaggctcctgcctggccctcaagagaactcagtccagagcagtgcctgtgggagacagcatctggagcccactggcaccattgacatgagggggcctgggcaagcagactgtgcagtggccataggcagaccattgggggaggtggtgaccctgagagtcctggaaagctccctcaactgctctgctggagatatgctgctcctctgggggaggctcacctggaggaaaatgtgtagaaaactgctggacatgaccttcagcagcaagaccaacaccctggtggtgaggcagaggtgtgggaggcctggtgggggtgtgctgcttaggtatggctcccagcttgctccagagaccttctacagagagtgtgacatgcagctctttgggccatggggggagattgtctccccatccctcagcccagccacctccaatgctgggggctgtaggctcttcatcaatgtggccccacatgcaaggattgccatccatgccctggccacaaacatgggggctgggacagagggggccaatgcctcctacatcctgataagggacacccacagcctcagaaccactgccttccatgggcagcaagtgctgtactgggaaagtgagagcagccaagctgagatggagttttctgaggggtttctgaaggcccaagcctcacttaggggccagtattggaccctgcagtcctgggttcctgaaatgcaagacccccagtcttggaaagggaaggaaggcacctgataagcggccgcaatcaaagcttgcctcgagcagcgctgctcgagagatctacgggtggcatccctgtgacccctccccagtgcctctcctggccctggaagttgccactccagtgcccaccagccttgtcctaataaaattaagttgcatcattttgtctgactaggtgtccttctataatattatggggtggaggggggtggtatggagcaaggggcaagttgggaagacaacctgtagggcctgcggggtctattgggaaccaagctggagtgcagtggcacaatcttggctcactgcaatctccgcctcctgggttcaagcgattctcctgcctcagcctcccgagttgttgggattccaggcatgcatgaccaggctcagctaatttttgtttttttggtagagacggggtttcaccatattggccaggctggtctccaactcctaatctcaggtgatctacccaccttggcctcccaaattgctgggattacaggcgtgaaccactgctcccttccctgtccttctgattttgtaggtaaccacgtgcggaccgagcggccgcaggaacccctagtgatggagttggccactccctctctgcgcgctcgctcgctcactgaggccgggcgaccaaaggtcgcccgacgcccgggctttgcccgggcggcctcagtgagcgagcgagcgcgcagctgcctgcagg

SEQ ID NO: 18 - DNA, 3834 bp, synthetic construct
  source 1..3834: mol_type = other DNA
gcacgcgtgtgtttgctgcttgcaatgtttgcccattttagggtggacacaggacgctgtggtttctgagccagggggcgactcagatcccagccagtggacttagcccctgtttgctcctccgataactggggtgaccttggttaatattcaccagcagcctcccccgttgcccctctggatccactgcttaaatacggacgaggacagggccctgtctcctcagcttcaggcaccaccactgacctgggacagtgaatccctcgaggggcgcgccgccaccatgcaccagcgtcacccccgggcaagatgccctcccctctgtgtggccggaatccttgcctgtggctttctcctgggctgctggggaccctcccatttccagcagagttgtcttcaggctttggagccacaggccgtgtcttcttacttgagccctggtgctcccttaaaaggccgccctccttcccctggcttccagaggcagaggcagaggcagaggcgggctgcaggcggcatcctacacctggagctgctggtggccgtgggccccgatgtcttccaggctcaccaggaggacacagagcgctatgtgctcaccaacctcaacatcggggcagaactgcttcgggacccgtccctgggggctcagtttcgggtgcacctggtgaagatggtcattctgacagagcctgagggtgctccaaatatcacagccaacctcacctcgtccctgctgagcgtctgtgggtggagccagaccatcaaccctgaggacgacacagatcctggccatgctgacctggtcctctatatcactaggtttgacctggagttgcctgatggtaaccggcaggtgcggggcgtcacccagctgggcggtgcctgctccccaacctggagctgcctcattaccgaggacactggcttcgacctgggagtcaccattgcccatgagattgggcacagcttcggcctggagcacgacggagcgcccggcagcggctgcggccccagcggacacgtgatggcttcggacggagctgctcctagagctggcctcgcttggtccccctgcagcagacggcagctgctgagcctgctcagcgcaggacgggcgcgctgcgtgtgggacccgccgcggcctcaacccgggtccgcggggcacccgccggatgcgcagcctggcctctactacagcgccaacgagcagtgccgcgtggccttcggccccaaggctgtcgcctgcaccttcgccagggagcacctggatatgtgccaggccctctcctgccacacagacccgctggaccaaagcagctgcagccgcctcctcgttcctctcctggatgggacagaatgtggcgtggagaagtggtgctccaagggtcgctgccgctccctggtggagctgacccccatagcagcagtgcatgggcgctggtctagctggggtccccgaagtccttgctcccgctcctgcggaggaggtgtggtcaccaggaggcggcagtgcaacaaccccagacctgcctttggggggcgtgcatgtgttggtgctgacctccaggccgagatgtgcaacactcaggcctgcgagaagacccagctggagttcatgtcgcaacagtgcgccaggaccgacggccagccgctgcgctcctcccctggcggcgcctccttctaccactggggtgctgctgtaccacacagccaaggggatgctctgtgcagacacatgtgccgggccattggcgagagcttcatcatgaagcgtggagacagcttcctcgatgggacccggtgtatgccaagtggcccccgggaggacgggaccctgagcctgtgtgtgtcgggcagctgcaggacatttggctgtgatggtaggatggactcccagcaggtatgggacaggtgccaggtgtgtggtggggacaacagcacgtgcagcccacggaagggctctttcacagctggcagagcgagagaatatgtcacgtttctgacagttacccccaacctgaccagtgtctacattgccaaccacaggcctctcttcacacacttggcggtgaggatcggagggcgctatgtcgtggctgggaagatgagcatctcccctaacaccacctacccctccctcctggaggatggtcgtgtcgagtacagagtggccctcaccgaggaccggctgccccgcctggaggagatccgcatctggggacccctccaggaagatgctgacatccaggtttacaggcggtatggcgaggagtatggcaacctcacccgcccagacatcaccttcacctacttccagcctaagccacggcaggcctgggtgtgggccgctgtgcgtgggccctgctcggtgagctgtggggcagggctgcgctgggtaaactacagctgcctggaccaggccaggaaggagttggtggagactgtccagtgccaagggagccagcagccaccagcgtggccagaggcctgcgtgctcgaaccctgccctccctactggaaagtcatgtcccttggcccatgttcggccagctgtggccttggcactgctagacgctcggtggcctgtgtgcagctcgaccaaggccaggacgtggaggtggacgaggcggcctgtgcggcgctggtgcggcccgaggccagtgtcccctgtctcattgccgactgcacctaccgctggcatgttggcacctggatggagtgctctgtttcctgtggggatggcatccagcgccggcgtgacacctgcctcggaccccaggcccaggcgcctgtgccagctgatttctgccagcacttgcccaagccggtgactgtgcgtggctgctgggctgggccctgtgtgggacagggtacgcccagcctggtgccccacgaagaagccgctgctccaggacggaccacagccacccctgctggtgcctccctggagtggtcccaggcccggggcctgctcttctccccggctccccagcctcggcggctcctgcccgggccccaggaaaactcagtgcagtccagtgcctgtggcaggcagcaccttgagccaacaggaaccattgacatgcgaggcccagggcaggcagactgtgcagtggccattgggcggcccctcggggaggtggtgaccctccgcgtccttgagagttctctcaactgcagtgcgggggacatgttgctgctttggggccggctcacctggaggaagatgtgcaggaagctgttggacatgactttcagctccaagaccaacacgctggtggtgaggcagcgctgcgggcggccaggaggtggggtgctgctgcggtatgggagccagcttgctcctgaaaccttctacagagaatgtgacatgcagctctttgggccctggggtgaaatcgtgagcccctcgctgagtccagccacgagtaatgcagggggctgccggctcttcattaatgtggctccgcacgcacggattgccatccatgccctggccaccaacatgggcgctgggaccgagggagccaatgccagctacatcttgatccgggacacccacagcttgaggaccacagcgtttcatgggcagcaggtgctctactgggagtcagagagcagccaggctgagatggagttcagcgagggcttcctgaaggctcaggccagcctgcggggccagtattggaccctccaatcatgggtaccggagatgcaggaccctcagtcctggaagggaaaggaaggaacctgataagcggccgcaatcaaagcttgagctcaataaaagatctttattttcattagatctgtgtgttggttttttgtgtg

SEQ ID NO: 19 - DNA, 4118 bp, synthetic construct
  source 1..4118: mol_type = other DNA
cctgcaggcagctgcgcgctcgctcgctcactgaggccgcccgggcgtcgggcgacctttggtcgcccggcctcagtgagcgagcgagcgcgcagagagggagtggccaactccatcactaggggttcctgcggccgcacgcgtggagctagttattaatagtaatcaattacggggtcattagttcatagcccatatatggagttccgcgttacataacttacggtaaatggcccgcctggctgaccgcccaacgacccccgcccattgacgtcaataatgacgtatgttcccatagtaacgtcaatagggactttccattgacgtcaatgggtggagtatttacggtaaactgcccacttggcagtacatcaagtgtatcatatgccaagtacgccccctattgacgtcaatgacggtaaatggcccgcctggcattatgcccagtacatgaccttatgggactttcctacttggcagtacatctacgtattagtcatcgctattaccatggtgatgcggttttggcagtacatcaatgggcgtggatagcggtttgactcacggggatttccaagtctccaccccattgacgtcaatgggagtttgttttgcaccaaaatcaacgggactttccaaaatgtcgtaacaactccgccccattgacgcaaatgggcggtaggcgtgtacggtgggaggtctatataagcagagctcgtttagtgaaccgtcagatcgcctggagacgccatccacgctgttttgacctccatagaagacaccgggaccgatccagcctccgcggattcgaatcccggccgggaacggtgcattggaacgcggattccccgtgccaagagtgacgtaagtaccgcctatagagtctataggcccacaaaaaatgctttcttcttttaatatacttttttgtttatcttatttctaatactttccctaatctctttctttcagggcaataatgatacaatgtatcatgcctctttgcaccattctaaagaataacagtgataatttctgggttaaggcaatagcaatatttctgcatataaatatttctgcatataaattgtaactgatgtaagaggtttcatattgctaatagcagctacaatccagctaccattctgcttttattttatggttgggataaggctggattattctgagtccaagctaggcccttttgctaatcatgttcatacctcttatcttcctcccacagctcctgggcaacgtgctggtctgtgtgctggcccatcactttggcaaagaattgggattcgaacatcgattgaattcgaattggatcctcgaggggcgcgccgccaccatgcaccagcgtcacccccgggcaagatgccctcccctctgtgtggccggaatccttgcctgtggctttctcctgggctgctggggaccctcccatttccagcagagttgtcttcaggctttggagccacaggccgtgtcttcttacttgagccctggtgctcccttaaaaggccgccctccttcccctggcttccagaggcagaggcagaggcagaggcgggctgcaggcggcatcctacacctggagctgctggtggccgtgggccccgatgtcttccaggctcaccaggaggacacagagcgctatgtgctcaccaacctcaacatcggggcagaactgcttcgggacccgtccctgggggctcagtttcgggtgcacctggtgaagatggtcattctgacagagcctgagggtgctccaaatatcacagccaacctcacctcgtccctgctgagcgtctgtgggtggagccagaccatcaaccctgaggacgacacagatcctggccatgctgacctggtcctctatatcactaggtttgacctggagttgcctgatggtaaccggcaggtgcggggcgtcacccagctgggcggtgcctgctccccaacctggagctgcctcattaccgaggacactggcttcgacctgggagtcaccattgcccatgagattgggcacagcttcggcctggagcacgacggagcgcccggcagcggctgcggccccagcggacacgtgatggcttcggacggagctgctcctagagctggcctcgcttggtccccctgcagcagacggcagctgctgagcctgctcagcgcaggacgggcgcgctgcgtgtgggacccgccgcggcctcaacccgggtccgcggggcacccgccggatgcgcagcctggcctctactacagcgccaacgagcagtgccgcgtggccttcggccccaaggctgtcgcctgcaccttcgccagggagcacctggatatgtgccaggccctctcctgccacacagacccgctggaccaaagcagctgcagccgcctcctcgttcctctcctggatgggacagaatgtggcgtggagaagtggtgctccaagggtcgctgccgctccctggtggagctgacccccatagcagcagtgcatgggcgctggtctagctggggtccccgaagtccttgctcccgctcctgcggaggaggtgtggtcaccaggaggcggcagtgcaacaaccccagacctgcctttggggggcgtgcatgtgttggtgctgacctccaggccgagatgtgcaacactcaggcctgcgagaagacccagctggagttcatgtcgcaacagtgcgccaggaccgacggccagccgctgcgctcctcccctggcggcgcctccttctaccactggggtgctgctgtaccacacagccaaggggatgctctgtgcagacacatgtgccgggccattggcgagagcttcatcatgaagcgtggagacagcttcctcgatgggacccggtgtatgccaagtggcccccgggaggacgggaccctgagcctgtgtgtgtcgggcagctgcaggacatttggctgtgatggtaggatggactcccagcaggtatgggacaggtgccaggtgtgtggtggggacaacagcacgtgcagcccacggaagggctctttcacagctggcagagcgagagaatatgtcacgtttctgacagttacccccaacctgaccagtgtctacattgccaaccacaggcctctcttcacacacttggcggtgaggatcggagggcgctatgtcgtggctgggaagatgagcatctcccctaacaccacctacccctccctcctggaggatggtcgtgtcgagtacagagtggccctcaccgaggaccggctgccccgcctggaggagatccgcatctggggacccctccaggaagatgctgacatccaggtttacaggcggtatggcgaggagtatggcaacctcacccgcccagacatcaccttcacctacttccagcctaagccacggcaggcctgataagcggccgcaatcaaagcttgcctcgagcagcgctgctcgagagatctacgggtggcatccctgtgacccctccccagtgcctctcctggccctggaagttgccactccagtgcccaccagccttgtcctaataaaattaagttgcatcattttgtctgactaggtgtccttctataatattatggggtggaggggggtggtatggagcaaggggcaagttgggaagacaacctgtagggcctgcggggtctattgggaaccaagctggagtgcagtggcacaatcttggctcactgcaatctccgcctcctgggttcaagcgattctcctgcctcagcctcccgagttgttgggattccaggcatgcatgaccaggctcagctaatttttgtttttttggtagagacggggtttcaccatattggccaggctggtctccaactcctaatctcaggtgatctacccaccttggcctcccaaattgctgggattacaggcgtgaaccactgctcccttccctgtccttctgattttgtaggtaaccacgtgcggaccgagcggccgcaggaacccctagtgatggagttggccactccctctctgcgcgctcgctcgctcactgaggccgggcgaccaaaggtcgcccgacgcccgggctttgcccgggcggcctcagtgagcgagcgagcgcgcagctgcctgcagg

SEQ ID NO: 20 - DNA, 2717 bp, synthetic construct
  source 1..2717: mol_type = other DNA
cctgcaggcagctgcgcgctcgctcgctcactgaggccgcccgggcgtcgggcgacctttggtcgcccggcctcagtgagcgagcgagcgcgcagagagggagtggccaactccatcactaggggttcctgcggccgcacgcgtgtgtttgctgcttgcaatgtttgcccattttagggtggacacaggacgctgtggtttctgagccagggggcgactcagatcccagccagtggacttagcccctgtttgctcctccgataactggggtgaccttggttaatattcaccagcagcctcccccgttgcccctctggatccactgcttaaatacggacgaggacagggccctgtctcctcagcttcaggcaccaccactgacctgggacagtgaatccctcgaggggcgcgccgccaccatgcaccagcgtcacccccgggcaagatgccctcccctctgtgtggccggaatccttgcctgtggctttctcctgggctgctggggaccctcccatttccagcagagttgtcttcaggctttggagccacaggccgtgtcttcttacttgagccctggtgctcccttaaaaggccgccctccttcccctggcttccagaggcagaggcagaggcagaggcgggctgcaggcggcatcctacacctggagctgctggtggccgtgggccccgatgtcttccaggctcaccaggaggacacagagcgctatgtgctcaccaacctcaacatcggggcagaactgcttcgggacccgtccctgggggctcagtttcgggtgcacctggtgaagatggtcattctgacagagcctgagggtgctccaaatatcacagccaacctcacctcgtccctgctgagcgtctgtgggtggagccagaccatcaaccctgaggacgacacagatcctggccatgctgacctggtcctctatatcactaggtttgacctggagttgcctgatggtaaccggcaggtgcggggcgtcacccagctgggcggtgcctgctccccaacctggagctgcctcattaccgaggacactggcttcgacctgggagtcaccattgcccatgagattgggcacagcttcggcctggagcacgacggagcgcccggcagcggctgcggccccagcggacacgtgatggcttcggacggagctgctcctagagctggcctcgcttggtccccctgcagcagacggcagctgctgagcctgctcagcgcaggacgggcgcgctgcgtgtgggacccgccgcggcctcaacccgggtccgcggggcacccgccggatgcgcagcctggcctctactacagcgccaacgagcagtgccgcgtggccttcggccccaaggctgtcgcctgcaccttcgccagggagcacctggatatgtgccaggccctctcctgccacacagacccgctggaccaaagcagctgcagccgcctcctcgttcctctcctggatgggacagaatgtggcgtggagaagtggtgctccaagggtcgctgccgctccctggtggagctgacccccatagcagcagtgcatgggcgctggtctagctggggtccccgaagtccttgctcccgctcctgcggaggaggtgtggtcaccaggaggcggcagtgcaacaaccccagacctgcctttggggggcgtgcatgtgttggtgctgacctccaggccgagatgtgcaacactcaggcctgcgagaagacccagctggagttcatgtcgcaacagtgcgccaggaccgacggccagccgctgcgctcctcccctggcggcgcctccttctaccactggggtgctgctgtaccacacagccaaggggatgctctgtgcagacacatgtgccgggccattggcgagagcttcatcatgaagcgtggagacagcttcctcgatgggacccggtgtatgccaagtggcccccgggaggacgggaccctgagcctgtgtgtgtcgggcagctgcaggacatttggctgtgatggtaggatggactcccagcaggtatgggacaggtgccaggtgtgtggtggggacaacagcacgtgcagcccacggaagggctctttcacagctggcagagcgagagaatatgtcacgtttctgacagttacccccaacctgaccagtgtctacattgccaaccacaggcctctcttcacacacttggcggtgaggatcggagggcgctatgtcgtggctgggaagatgagcatctcccctaacaccacctacccctccctcctggaggatggtcgtgtcgagtacagagtggccctcaccgaggaccggctgccccgcctggaggagatccgcatctggggacccctccaggaagatgctgacatccaggtttacaggcggtatggcgaggagtatggcaacctcacccgcccagacatcaccttcacctacttccagcctaagccacggcaggcctgataagcggccgcaatcaaagcttgagctcaataaaagatctttattttcattagatctgtgtgttggttttttgtgtggtcgaccggaccgagcggccgcaggaacccctagtgatggagttggccactccctctctgcgcgctcgctcgctcactgaggccgggcgaccaaaggtcgcccgacgcccgggctttgcccgggcggcctcagtgagcgagcgagcgcgcagctgcctgcagg

SEQ ID NO: 21 - DNA, 4943 bp, synthetic construct
  source 1..4943: mol_type = other DNA
cctgcaggcagctgcgcgctcgctcgctcactgaggccgcccgggcgtcgggcgacctttggtcgcccggcctcagtgagcgagcgagcgcgcagagagggagtggccaactccatcactaggggttcctgcggccgcacgcgtgtgtttgctgcttgcaatgtttgcccattttagggtggacacaggacgctgtggtttctgagccagggggcgactcagatcccagccagtggacttagcccctgtttgctcctccgataactggggtgaccttggttaatattcaccagcagcctcccccgttgcccctctggatccactgcttaaatacggacgaggacagggccctgtctcctcagcttcaggcaccaccactgacctgggacagtgaatccctcgaggggcgcgccgccaccatgcaccagcgtcacccccgggcaagatgccctcccctctgtgtggccggaatccttgcctgtggctttctcctgggctgctggggaccctcccatttccagcagagttgtcttcaggctttggagccacaggccgtgtcttcttacttgagccctggtgctcccttaaaaggccgccctccttcccctggcttccagaggcagaggcagaggcagaggcgggctgcaggcggcatcctacacctggagctgctggtggccgtgggccccgatgtcttccaggctcaccaggaggacacagagcgctatgtgctcaccaacctcaacatcggggcagaactgcttcgggacccgtccctgggggctcagtttcgggtgcacctggtgaagatggtcattctgacagagcctgagggtgctccaaatatcacagccaacctcacctcgtccctgctgagcgtctgtgggtggagccagaccatcaaccctgaggacgacacagatcctggccatgctgacctggtcctctatatcactaggtttgacctggagttgcctgatggtaaccggcaggtgcggggcgtcacccagctgggcggtgcctgctccccaacctggagctgcctcattaccgaggacactggcttcgacctgggagtcaccattgcccatgagattgggcacagcttcggcctggagcacgacggagcgcccggcagcggctgcggccccagcggacacgtgatggcttcggacggagctgctcctagagctggcctcgcttggtccccctgcagcagacggcagctgctgagcctgctcagcgcaggacgggcgcgctgcgtgtgggacccgccgcggcctcaacccgggtccgcggggcacccgccggatgcgcagcctggcctctactacagcgccaacgagcagtgccgcgtggccttcggccccaaggctgtcgcctgcaccttcgccagggagcacctggatatgtgccaggccctctcctgccacacagacccgctggaccaaagcagctgcagccgcctcctcgttcctctcctggatgggacagaatgtggcgtggagaagtggtgctccaagggtcgctgccgctccctggtggagctgacccccatagcagcagtgcatgggcgctggtctagctggggtccccgaagtccttgctcccgctcctgcggaggaggtgtggtcaccaggaggcggcagtgcaacaaccccagacctgcctttggggggcgtgcatgtgttggtgctgacctccaggccgagatgtgcaacactcaggcctgcgagaagacccagctggagttcatgtcgcaacagtgcgccaggaccgacggccagccgctgcgctcctcccctggcggcgcctccttctaccactggggtgctgctgtaccacacagccaaggggatgctctgtgcagacacatgtgccgggccattggcgagagcttcatcatgaagcgtggagacagcttcctcgatgggacccggtgtatgccaagtggcccccgggaggacgggaccctgagcctgtgtgtgtcgggcagctgcaggacatttggctgtgatggtaggatggactcccagcaggtatgggacaggtgccaggtgtgtggtggggacaacagcacgtgcagcccacggaagggctctttcacagctggcagagcgagagaatatgtcacgtttctgacagttacccccaacctgaccagtgtctacattgccaaccacaggcctctcttcacacacttggcggtgaggatcggagggcgctatgtcgtggctgggaagatgagcatctcccctaacaccacctacccctccctcctggaggatggtcgtgtcgagtacagagtggccctcaccgaggaccggctgccccgcctggaggagatccgcatctggggacccctccaggaagatgctgacatccaggtttacaggcggtatggcgaggagtatggcaacctcacccgcccagacatcaccttcacctacttccagcctaagccacggcaggcctgggtgtgggccgctgtgcgtgggccctgctcggtgagctgtggggcagggctgcgctgggtaaactacagctgcctggaccaggccaggaaggagttggtggagactgtccagtgccaagggagccagcagccaccagcgtggccagaggcctgcgtgctcgaaccctgccctccctactgggcggtgggagacttcggcccatgcagcgcctcctgtgggggtggcctgcgggagcggccagtgcgctgcgtggaggcccagggcagcctcctgaagacattgcccccagcccggtgcagagcaggggcccagcagccagctgtggcgctggaaacctgcaacccccagccctgccctgccaggtgggaggtgtcagagcccagctcatgcacatcagctggtggagcaggcctggccttggagaacgagacctgtgtgccaggggcagatggcctggaggctccagtgactgaggggcctggctccgtagatgagaagctgcctgcccctgagccctgtgtcgggatgtcatgtcctccaggctggggccatctggatgccacctctgcaggggagaaggctccctccccttggggcagcatcaggacgggggctcaagctgcacacgtgtggacccctgcggcagggtcgtgctccgtctcctgcgggcgaggtctgatggagctgcgtttcctgtgcatggactctgccctcagggtgcctgtccaggaagagctgtgtggcctggcaagcaagcctgggagccggcgggaggtctgccaggctgtcccgtgccctgctcggtggcagtacaagctggcggcctgcagcgtgagctgtgggagaggggtcgtgcggagaatcctgtattgtgcccgggctcatggggaggacgatggtgaggagatcctgttggacacccagtgccaggggctgcctcgcccggaaccccaggaggcctgcagcctggagccctgcccacctaggtggaaagtcatgtcccttggcccatgttcggccagctgtggccttggcactgctagacgctcggtggcctgtgtgcagctcgaccaaggccaggacgtggaggtggacgaggcggcctgtgcggcgctggtgcggcccgaggccagtgtcccctgtctcattgccgactgcacctaccgctggcatgttggcacctggatggagtgctctgtttcctgtggggatggcatccagcgccggcgtgacacctgcctcggaccccaggcccaggcgcctgtgccagctgatttctgccagcacttgcccaagccggtgactgtgcgtggctgctgggctgggccctgtgtgggacagggtacgcccagcctggtgccccacgaagaagccgctgctccaggacggaccacagccacccctgctggtgcctccctggagtggtcccaggcccggggcctgctcttctccccggctccccagcctcggcggctcctgcccgggccccaggaaaactcagtgcagtccagtgcctgtggcaggcagcaccttgagccaacaggaaccattgacatgcgaggcccagggcaggcagactgtgcagtggccattgggcggcccctcggggaggtggtgaccctccgcgtccttgagagttctctcaactgcagtgcgggggacatgttgctgctttggggccggctcacctggaggaagatgtgcaggaagctgttggacatgactttcagctccaagaccaacacgctggtggtgaggcagcgctgcgggcggccaggaggtggggtgctgctgcggtatgggagccagcttgctcctgaaaccttctacagagaatgtgacatgcagctctttgggccctggggtgaaatcgtgagcccctcgctgagtccagccacgagtaatgcagggggctgccggctcttcattaatgtggctccgcacgcacggattgccatccatgccctggccaccaacatgggcgctgggaccgagggagccaatgccagctacatcttgatccgggacacccacagcttgaggaccacagcgtttcatgggcagcaggtgctctactgggagtcagagagcagccaggctgagatggagttcagcgagggcttcctgaaggctcaggccagcctgcggggccagtattggaccctccaatcatgggtaccggagatgcaggaccctcagtcctggaagggaaaggaaggaacctgataagcggccgcaatcaaagcttgagctcaataaaagatctttattttcattagatctgtgtgttggttttttgtgtggtcgaccggaccgagcggccgcaggaacccctagtgatggagttggccactccctctctgcgcgctcgctcgctcactgaggccgggcgaccaaaggtcgcccgacgcccgggctttgcccgggcggcctcagtgagcgagcgagcgcgcagctgcctgcagg

SEQ ID NO: 22 - DNA, 5534 bp, synthetic construct
  source 1..5534: mol_type = other DNA
cctgcaggcagctgcgcgctcgctcgctcactgaggccgcccgggcgtcgggcgacctttggtcgcccggcctcagtgagcgagcgagcgcgcagagagggagtggccaactccatcactaggggttcctgcggccgcacgcgtggagctagttattaatagtaatcaattacggggtcattagttcatagcccatatatggagttccgcgttacataacttacggtaaatggcccgcctggctgaccgcccaacgacccccgcccattgacgtcaataatgacgtatgttcccatagtaacgtcaatagggactttccattgacgtcaatgggtggagtatttacggtaaactgcccacttggcagtacatcaagtgtatcatatgccaagtacgccccctattgacgtcaatgacggtaaatggcccgcctggcattatgcccagtacatgaccttatgggactttcctacttggcagtacatctacgtattagtcatcgctattaccatggtgatgcggttttggcagtacatcaatgggcgtggatagcggtttgactcacggggatttccaagtctccaccccattgacgtcaatgggagtttgttttgcaccaaaatcaacgggactttccaaaatgtcgtaacaactccgccccattgacgcaaatgggcggtaggcgtgtacggtgggaggtctatataagcagagctcgtttagtgaaccgtcagatcgcctggagacgccatccacgctgttttgacctccatagaagacaccgggaccgatccagcctccgcggattcgaatcccggccgggaacggtgcattggaacgcggattccccgtgccaagagtgacgtaagtaccgcctatagagtctataggcccacaaaaaatgctttcttcttttaatatacttttttgtttatcttatttctaatactttccctaatctctttctttcagggcaataatgatacaatgtatcatgcctctttgcaccattctaaagaataacagtgataatttctgggttaaggcaatagcaatatttctgcatataaatatttctgcatataaattgtaactgatgtaagaggtttcatattgctaatagcagctacaatccagctaccattctgcttttattttatggttgggataaggctggattattctgagtccaagctaggcccttttgctaatcatgttcatacctcttatcttcctcccacagctcctgggcaacgtgctggtctgtgtgctggcccatcactttggcaaagaattgggattcgaacatcgattgaattcgaattggatcctcgaggggcgcgccgccaccatgcaccagcgtcacccccgggcaagatgccctcccctctgtgtggccggaatccttgcctgtggctttctcctgggctgctggggaccctcccatttccagcagagttgtcttcaggctttggagccacaggccgtgtcttcttacttgagccctggtgctcccttaaaaggccgccctccttcccctggcttccagaggcagaggcagaggcagaggcgggctgcaggcggcatcctacacctggagctgctggtggccgtgggccccgatgtcttccaggctcaccaggaggacacagagcgctatgtgctcaccaacctcaacatcggggcagaactgcttcgggacccgtccctgggggctcagtttcgggtgcacctggtgaagatggtcattctgacagagcctgagggtgctccaaatatcacagccaacctcacctcgtccctgctgagcgtctgtgggtggagccagaccatcaaccctgaggacgacacagatcctggccatgctgacctggtcctctatatcactaggtttgacctggagttgcctgatggtaaccggcaggtgcggggcgtcacccagctgggcggtgcctgctccccaacctggagctgcctcattaccgaggacactggcttcgacctgggagtcaccattgcccatgagattgggcacagcttcggcctggagcacgacggagcgcccggcagcggctgcggccccagcggacacgtgatggcttcggacggagctgctcctagagctggcctcgcttggtccccctgcagcagacggcagctgctgagcctgctcagcgcaggacgggcgcgctgcgtgtgggacccgccgcggcctcaacccgggtccgcggggcacccgccggatgcgcagcctggcctctactacagcgccaacgagcagtgccgcgtggccttcggccccaaggctgtcgcctgcaccttcgccagggagcacctggatatgtgccaggccctctcctgccacacagacccgctggaccaaagcagctgcagccgcctcctcgttcctctcctggatgggacagaatgtggcgtggagaagtggtgctccaagggtcgctgccgctccctggtggagctgacccccatagcagcagtgcatgggcgctggtctagctggggtccccgaagtccttgctcccgctcctgcggaggaggtgtggtcaccaggaggcggcagtgcaacaaccccagacctgcctttggggggcgtgcatgtgttggtgctgacctccaggccgagatgtgcaacactcaggcctgcgagaagacccagctggagttcatgtcgcaacagtgcgccaggaccgacggccagccgctgcgctcctcccctggcggcgcctccttctaccactggggtgctgctgtaccacacagccaaggggatgctctgtgcagacacatgtgccgggccattggcgagagcttcatcatgaagcgtggagacagcttcctcgatgggacccggtgtatgccaagtggcccccgggaggacgggaccctgagcctgtgtgtgtcgggcagctgcaggacatttggctgtgatggtaggatggactcccagcaggtatgggacaggtgccaggtgtgtggtggggacaacagcacgtgcagcccacggaagggctctttcacagctggcagagcgagagaatatgtcacgtttctgacagttacccccaacctgaccagtgtctacattgccaaccacaggcctctcttcacacacttggcggtgaggatcggagggcgctatgtcgtggctgggaagatgagcatctcccctaacaccacctacccctccctcctggaggatggtcgtgtcgagtacagagtggccctcaccgaggaccggctgccccgcctggaggagatccgcatctggggacccctccaggaagatgctgacatccaggtttacaggcggtatggcgaggagtatggcaacctcacccgcccagacatcaccttcacctacttccagcctaagccacggcaggcctgggtgtgggccgctgtgcgtgggccctgctcggtgagctgtggggcagggctgcgctgggtaaactacagctgcctggaccaggccaggaaggagttggtggagactgtccagtgccaagggagccagcagccaccagcgtggccagaggcctgcgtgctcgaaccctgccctccctactggaaagtcatgtcccttggcccatgttcggccagctgtggccttggcactgctagacgctcggtggcctgtgtgcagctcgaccaaggccaggacgtggaggtggacgaggcggcctgtgcggcgctggtgcggcccgaggccagtgtcccctgtctcattgccgactgcacctaccgctggcatgttggcacctggatggagtgctctgtttcctgtggggatggcatccagcgccggcgtgacacctgcctcggaccccaggcccaggcgcctgtgccagctgatttctgccagcacttgcccaagccggtgactgtgcgtggctgctgggctgggccctgtgtgggacagggtacgcccagcctggtgccccacgaagaagccgctgctccaggacggaccacagccacccctgctggtgcctccctggagtggtcccaggcccggggcctgctcttctccccggctccccagcctcggcggctcctgcccgggccccaggaaaactcagtgcagtccagtgcctgtggcaggcagcaccttgagccaacaggaaccattgacatgcgaggcccagggcaggcagactgtgcagtggccattgggcggcccctcggggaggtggtgaccctccgcgtccttgagagttctctcaactgcagtgcgggggacatgttgctgctttggggccggctcacctggaggaagatgtgcaggaagctgttggacatgactttcagctccaagaccaacacgctggtggtgaggcagcgctgcgggcggccaggaggtggggtgctgctgcggtatgggagccagcttgctcctgaaaccttctacagagaatgtgacatgcagctctttgggccctggggtgaaatcgtgagcccctcgctgagtccagccacgagtaatgcagggggctgccggctcttcattaatgtggctccgcacgcacggattgccatccatgccctggccaccaacatgggcgctgggaccgagggagccaatgccagctacatcttgatccgggacacccacagcttgaggaccacagcgtttcatgggcagcaggtgctctactgggagtcagagagcagccaggctgagatggagttcagcgagggcttcctgaaggctcaggccagcctgcggggccagtattggaccctccaatcatgggtaccggagatgcaggaccctcagtcctggaagggaaaggaaggaacctgataagcggccgcaatcaaagcttgcctcgagcagcgctgctcgagagatctacgggtggcatccctgtgacccctccccagtgcctctcctggccctggaagttgccactccagtgcccaccagccttgtcctaataaaattaagttgcatcattttgtctgactaggtgtccttctataatattatggggtggaggggggtggtatggagcaaggggcaagttgggaagacaacctgtagggcctgcggggtctattgggaaccaagctggagtgcagtggcacaatcttggctcactgcaatctccgcctcctgggttcaagcgattctcctgcctcagcctcccgagttgttgggattccaggcatgcatgaccaggctcagctaatttttgtttttttggtagagacggggtttcaccatattggccaggctggtctccaactcctaatctcaggtgatctacccaccttggcctcccaaattgctgggattacaggcgtgaaccactgctcccttccctgtccttctgattttgtaggtaaccacgtgcggaccgagcggccgcaggaacccctagtgatggagttggccactccctctctgcgcgctcgctcgctcactgaggccgggcgaccaaaggtcgcccgacgcccgggctttgcccgggcggcctcagtgagcgagcgagcgcgcagctgcctgcagg

SEQ ID NO: 23 - DNA, 5957 bp, synthetic construct
  source 1..5957: mol_type = other DNA
cctgcaggcagctgcgcgctcgctcgctcactgaggccgcccgggcgtcgggcgacctttggtcgcccggcctcagtgagcgagcgagcgcgcagagagggagtggccaactccatcactaggggttcctgcggccgcacgcgtggagctagttattaatagtaatcaattacggggtcattagttcatagcccatatatggagttccgcgttacataacttacggtaaatggcccgcctggctgaccgcccaacgacccccgcccattgacgtcaataatgacgtatgttcccatagtaacgtcaatagggactttccattgacgtcaatgggtggagtatttacggtaaactgcccacttggcagtacatcaagtgtatcatatgccaagtacgccccctattgacgtcaatgacggtaaatggcccgcctggcattatgcccagtacatgaccttatgggactttcctacttggcagtacatctacgtattagtcatcgctattaccatggtgatgcggttttggcagtacatcaatgggcgtggatagcggtttgactcacggggatttccaagtctccaccccattgacgtcaatgggagtttgttttgcaccaaaatcaacgggactttccaaaatgtcgtaacaactccgccccattgacgcaaatgggcggtaggcgtgtacggtgggaggtctatataagcagagctcgtttagtgaaccgtcagatcgcctggagacgccatccacgctgttttgacctccatagaagacaccgggaccgatccagcctccgcggattcgaatcccggccgggaacggtgcattggaacgcggattccccgtgccaagagtgacgtaagtaccgcctatagagtctataggcccacaaaaaatgctttcttcttttaatatacttttttgtttatcttatttctaatactttccctaatctctttctttcagggcaataatgatacaatgtatcatgcctctttgcaccattctaaagaataacagtgataatttctgggttaaggcaatagcaatatttctgcatataaatatttctgcatataaattgtaactgatgtaagaggtttcatattgctaatagcagctacaatccagctaccattctgcttttattttatggttgggataaggctggattattctgagtccaagctaggcccttttgctaatcatgttcatacctcttatcttcctcccacagctcctgggcaacgtgctggtctgtgtgctggcccatcactttggcaaagaattgggattcgaacatcgattgaattcgaattggatcctcgaggggcgcgccgccaccatgcaccagcgtcacccccgggcaagatgccctcccctctgtgtggccggaatccttgcctgtggctttctcctgggctgctggggaccctcccatttccagcagagttgtcttcaggctttggagccacaggccgtgtcttcttacttgagccctggtgctcccttaaaaggccgccctccttcccctggcttccagaggcagaggcagaggcagaggcgggctgcaggcggcatcctacacctggagctgctggtggccgtgggccccgatgtcttccaggctcaccaggaggacacagagcgctatgtgctcaccaacctcaacatcggggcagaactgcttcgggacccgtccctgggggctcagtttcgggtgcacctggtgaagatggtcattctgacagagcctgagggtgctccaaatatcacagccaacctcacctcgtccctgctgagcgtctgtgggtggagccagaccatcaaccctgaggacgacacagatcctggccatgctgacctggtcctctatatcactaggtttgacctggagttgcctgatggtaaccggcaggtgcggggcgtcacccagctgggcggtgcctgctccccaacctggagctgcctcattaccgaggacactggcttcgacctgggagtcaccattgcccatgagattgggcacagcttcggcctggagcacgacggagcgcccggcagcggctgcggccccagcggacacgtgatggcttcggacggagctgctcctagagctggcctcgcttggtccccctgcagcagacggcagctgctgagcctgctcagcgcaggacgggcgcgctgcgtgtgggacccgccgcggcctcaacccgggtccgcggggcacccgccggatgcgcagcctggcctctactacagcgccaacgagcagtgccgcgtggccttcggccccaaggctgtcgcctgcaccttcgccagggagcacctggatatgtgccaggccctctcctgccacacagacccgctggaccaaagcagctgcagccgcctcctcgttcctctcctggatgggacagaatgtggcgtggagaagtggtgctccaagggtcgctgccgctccctggtggagctgacccccatagcagcagtgcatgggcgctggtctagctggggtccccgaagtccttgctcccgctcctgcggaggaggtgtggtcaccaggaggcggcagtgcaacaaccccagacctgcctttggggggcgtgcatgtgttggtgctgacctccaggccgagatgtgcaacactcaggcctgcgagaagacccagctggagttcatgtcgcaacagtgcgccaggaccgacggccagccgctgcgctcctcccctggcggcgcctccttctaccactggggtgctgctgtaccacacagccaaggggatgctctgtgcagacacatgtgccgggccattggcgagagcttcatcatgaagcgtggagacagcttcctcgatgggacccggtgtatgccaagtggcccccgggaggacgggaccctgagcctgtgtgtgtcgggcagctgcaggacatttggctgtgatggtaggatggactcccagcaggtatgggacaggtgccaggtgtgtggtggggacaacagcacgtgcagcccacggaagggctctttcacagctggcagagcgagagaatatgtcacgtttctgacagttacccccaacctgaccagtgtctacattgccaaccacaggcctctcttcacacacttggcggtgaggatcggagggcgctatgtcgtggctgggaagatgagcatctcccctaacaccacctacccctccctcctggaggatggtcgtgtcgagtacagagtggccctcaccgaggaccggctgccccgcctggaggagatccgcatctggggacccctccaggaagatgctgacatccaggtttacaggcggtatggcgaggagtatggcaacctcacccgcccagacatcaccttcacctacttccagcctaagccacggcaggcctgggtgtgggccgctgtgcgtgggccctgctcggtgagctgtggggcagggctgcgctgggtaaactacagctgcctggaccaggccaggaaggagttggtggagactgtccagtgccaagggagccagcagccaccagcgtggccagaggcctgcgtgctcgaaccctgccctccctactgggcggtgggagacttcggcccatgcagcgcctcctgtgggggtggcctgcgggagcggccagtgcgctgcgtggaggcccagggcagcctcctgaagacattgcccccagcccggtgcagagcaggggcccagcagccagctgtggcgctggaaacctgcaacccccagccctgccctgccaggtgggaggtgtcagagcccagctcatgcacatcagctggtggagcaggcctggccttggagaacgagacctgtgtgccaggggcagatggcctggaggctccagtgactgaggggcctggctccgtagatgagaagctgcctgcccctgagccctgtgtcgggatgtcatgtcctccaggctggggccatctggatgccacctctgcaggggagaaggctccctccccttggggcagcatcaggacgggggctcaagctgcacacgtgtggacccctgcggcagggtcgtgctccgtctcctgcgggcgaggtctgatggagctgcgtttcctgtgcatggactctgccctcagggtgcctgtccaggaagagctgtgtggcctggcaagcaagcctgggagccggcgggaggtctgccaggctgtcccgtgccctgctcggtggcagtacaagctggcggcctgcagcgtgagctgtgggagaggggtcgtgcggagaatcctgtattgtgcccgggctcatggggaggacgatggtgaggagatcctgttggacacccagtgccaggggctgcctcgcccggaaccccaggaggcctgcagcctggagccctgcccacctaggtggaaagtcatgtcccttggcccatgttcggccagctgtggccttggcactgctagacgctcggtggcctgtgtgcagctcgaccaaggccaggacgtggaggtggacgaggcggcctgtgcggcgctggtgcggcccgaggccagtgtcccctgtctcattgccgactgcacctaccgctggcatgttggcacctggatggagtgctctgtttcctgtggggatggcatccagcgccggcgtgacacctgcctcggaccccaggcccaggcgcctgtgccagctgatttctgccagcacttgcccaagccggtgactgtgcgtggctgctgggctgggccctgtgtgggacagggtacgcccagcctggtgccccacgaagaagccgctgctccaggacggaccacagccacccctgctggtgcctccctggagtggtcccaggcccggggcctgctcttctccccggctccccagcctcggcggctcctgcccgggccccaggaaaactcagtgcagtccagtgcctgtggcaggcagcaccttgagccaacaggaaccattgacatgcgaggcccagggcaggcagactgtgcagtggccattgggcggcccctcggggaggtggtgaccctccgcgtccttgagagttctctcaactgcagtgcgggggacatgttgctgctttggggccggctcacctggaggaagatgtgcaggaagctgttggacatgactttcagctccaagaccaacacgctggtggtgaggcagcgctgcgggcggccaggaggtggggtgctgctgcggtatgggagccagcttgctcctgaaaccttctacagagaatgataagcggccgcaatcaaagcttgcctcgagcagcgctgctcgagagatctacgggtggcatccctgtgacccctccccagtgcctctcctggccctggaagttgccactccagtgcccaccagccttgtcctaataaaattaagttgcatcattttgtctgactaggtgtccttctataatattatggggtggaggggggtggtatggagcaaggggcaagttgggaagacaacctgtagggcctgcggggtctattgggaaccaagctggagtgcagtggcacaatcttggctcactgcaatctccgcctcctgggttcaagcgattctcctgcctcagcctcccgagttgttgggattccaggcatgcatgaccaggctcagctaatttttgtttttttggtagagacggggtttcaccatattggccaggctggtctccaactcctaatctcaggtgatctacccaccttggcctcccaaattgctgggattacaggcgtgaaccactgctcccttccctgtccttctgattttgtaggtaaccacgtgcggaccgagcggccgcaggaacccctagtgatggagttggccactccctctctgcgcgctcgctcgctcactgaggccgggcgaccaaaggtcgcccgacgcccgggctttgcccgggcggcctcagtgagcgagcgagcgcgcagctgcctgcagg

SEQ ID NO: 24 - DNA, 5147 bp, synthetic construct
  source 1..5147: mol_type = other DNA
cctgcaggcagctgcgcgctcgctcgctcactgaggccgcccgggcgtcgggcgacctttggtcgcccggcctcagtgagcgagcgagcgcgcagagagggagtggccaactccatcactaggggttcctgcggccgcacgcgtggagctagttattaatagtaatcaattacggggtcattagttcatagcccatatatggagttccgcgttacataacttacggtaaatggcccgcctggctgaccgcccaacgacccccgcccattgacgtcaataatgacgtatgttcccatagtaacgtcaatagggactttccattgacgtcaatgggtggagtatttacggtaaactgcccacttggcagtacatcaagtgtatcatatgccaagtacgccccctattgacgtcaatgacggtaaatggcccgcctggcattatgcccagtacatgaccttatgggactttcctacttggcagtacatctacgtattagtcatcgctattaccatggtgatgcggttttggcagtacatcaatgggcgtggatagcggtttgactcacggggatttccaagtctccaccccattgacgtcaatgggagtttgttttgcaccaaaatcaacgggactttccaaaatgtcgtaacaactccgccccattgacgcaaatgggcggtaggcgtgtacggtgggaggtctatataagcagagctcgtttagtgaaccgtcagatcgcctggagacgccatccacgctgttttgacctccatagaagacaccgggaccgatccagcctccgcggattcgaatcccggccgggaacggtgcattggaacgcggattccccgtgccaagagtgacgtaagtaccgcctatagagtctataggcccacaaaaaatgctttcttcttttaatatacttttttgtttatcttatttctaatactttccctaatctctttctttcagggcaataatgatacaatgtatcatgcctctttgcaccattctaaagaataacagtgataatttctgggttaaggcaatagcaatatttctgcatataaatatttctgcatataaattgtaactgatgtaagaggtttcatattgctaatagcagctacaatccagctaccattctgcttttattttatggttgggataaggctggattattctgagtccaagctaggcccttttgctaatcatgttcatacctcttatcttcctcccacagctcctgggcaacgtgctggtctgtgtgctggcccatcactttggcaaagaattgggattcgaacatcgattgaattcgaattggatcctcgaggggcgcgccgccaccatgcaccagcgtcacccccgggcaagatgccctcccctctgtgtggccggaatccttgcctgtggctttctcctgggctgctggggaccctcccatttccagcagagttgtcttcaggctttggagccacaggccgtgtcttcttacttgagccctggtgctcccttaaaaggccgccctccttcccctggcttccagaggcagaggcagaggcagaggcgggctgcaggcggcatcctacacctggagctgctggtggccgtgggccccgatgtcttccaggctcaccaggaggacacagagcgctatgtgctcaccaacctcaacatcggggcagaactgcttcgggacccgtccctgggggctcagtttcgggtgcacctggtgaagatggtcattctgacagagcctgagggtgctccaaatatcacagccaacctcacctcgtccctgctgagcgtctgtgggtggagccagaccatcaaccctgaggacgacacagatcctggccatgctgacctggtcctctatatcactaggtttgacctggagttgcctgatggtaaccggcaggtgcggggcgtcacccagctgggcggtgcctgctccccaacctggagctgcctcattaccgaggacactggcttcgacctgggagtcaccattgcccatgagattgggcacagcttcggcctggagcacgacggagcgcccggcagcggctgcggccccagcggacacgtgatggcttcggacggagctgctcctagagctggcctcgcttggtccccctgcagcagacggcagctgctgagcctgctcagcgcaggacgggcgcgctgcgtgtgggacccgccgcggcctcaacccgggtccgcggggcacccgccggatgcgcagcctggcctctactacagcgccaacgagcagtgccgcgtggccttcggccccaaggctgtcgcctgcaccttcgccagggagcacctggatatgtgccaggccctctcctgccacacagacccgctggaccaaagcagctgcagccgcctcctcgttcctctcctggatgggacagaatgtggcgtggagaagtggtgctccaagggtcgctgccgctccctggtggagctgacccccatagcagcagtgcatgggcgctggtctagctggggtccccgaagtccttgctcccgctcctgcggaggaggtgtggtcaccaggaggcggcagtgcaacaaccccagacctgcctttggggggcgtgcatgtgttggtgctgacctccaggccgagatgtgcaacactcaggcctgcgagaagacccagctggagttcatgtcgcaacagtgcgccaggaccgacggccagccgctgcgctcctcccctggcggcgcctccttctaccactggggtgctgctgtaccacacagccaaggggatgctctgtgcagacacatgtgccgggccattggcgagagcttcatcatgaagcgtggagacagcttcctcgatgggacccggtgtatgccaagtggcccccgggaggacgggaccctgagcctgtgtgtgtcgggcagctgcaggacatttggctgtgatggtaggatggactcccagcaggtatgggacaggtgccaggtgtgtggtggggacaacagcacgtgcagcccacggaagggctctttcacagctggcagagcgagagaatatgtcacgtttctgacagttacccccaacctgaccagtgtctacattgccaaccacaggcctctcttcacacacttggcggtgaggatcggagggcgctatgtcgtggctgggaagatgagcatctcccctaacaccacctacccctccctcctggaggatggtcgtgtcgagtacagagtggccctcaccgaggaccggctgccccgcctggaggagatccgcatctggggacccctccaggaagatgctgacatccaggtttacaggcggtatggcgaggagtatggcaacctcacccgcccagacatcaccttcacctacttccagcctaagccacggcaggcctgggtgtgggccgctgtgcgtgggccctgctcggtgagctgtggggcagggctgcgctgggtaaactacagctgcctggaccaggccaggaaggagttggtggagactgtccagtgccaagggagccagcagccaccagcgtggccagaggcctgcgtgctcgaaccctgccctccctactggaaagtcatgtcccttggcccatgttcggccagctgtggccttggcactgctagacgctcggtggcctgtgtgcagctcgaccaaggccaggacgtggaggtggacgaggcggcctgtgcggcgctggtgcggcccgaggccagtgtcccctgtctcattgccgactgcacctaccgctggcatgttggcacctggatggagtgctctgtttcctgtggggatggcatccagcgccggcgtgacacctgcctcggaccccaggcccaggcgcctgtgccagctgatttctgccagcacttgcccaagccggtgactgtgcgtggctgctgggctgggccctgtgtgggacagggtacgcccagcctggtgccccacgaagaagccgctgctccaggacggaccacagccacccctgctggtgcctccctggagtggtcccaggcccggggcctgctcttctccccggctccccagcctcggcggctcctgcccgggccccaggaaaactcagtgcagtccagtgcctgtggcaggcagcaccttgagccaacaggaaccattgacatgcgaggcccagggcaggcagactgtgcagtggccattgggcggcccctcggggaggtggtgaccctccgcgtccttgagagttctctcaactgcagtgcgggggacatgttgctgctttggggccggctcacctggaggaagatgtgcaggaagctgttggacatgactttcagctccaagaccaacacgctggtggtgaggcagcgctgcgggcggccaggaggtggggtgctgctgcggtatgggagccagcttgctcctgaaaccttctacagagaatgataagcggccgcaatcaaagcttgcctcgagcagcgctgctcgagagatctacgggtggcatccctgtgacccctccccagtgcctctcctggccctggaagttgccactccagtgcccaccagccttgtcctaataaaattaagttgcatcattttgtctgactaggtgtccttctataatattatggggtggaggggggtggtatggagcaaggggcaagttgggaagacaacctgtagggcctgcggggtctattgggaaccaagctggagtgcagtggcacaatcttggctcactgcaatctccgcctcctgggttcaagcgattctcctgcctcagcctcccgagttgttgggattccaggcatgcatgaccaggctcagctaatttttgtttttttggtagagacggggtttcaccatattggccaggctggtctccaactcctaatctcaggtgatctacccaccttggcctcccaaattgctgggattacaggcgtgaaccactgctcccttccctgtccttctgattttgtaggtaaccacgtgcggaccgagcggccgcaggaacccctagtgatggagttggccactccctctctgcgcgctcgctcgctcactgaggccgggcgaccaaaggtcgcccgacgcccgggctttgcccgggcggcctcagtgagcgagcgagcgcgcagctgcctgcagg

SEQ ID NO: 25 - DNA, 4401 bp, synthetic construct
  source 1..4401: mol_type = other DNA
tgcaggcagctgcgcgctcgctcgctcactgaggccgcccgggcaaagcccgggcgtcgggcgacctttggtcgcccggcctcagtgagcgagcgagcgcgcagagagggagtggccaactccatcactaggggttcctgatgcggctgcacgcgtgtgtttgctgcttgcaatgtttgcccattttagggtggacacaggacgctgtggtttctgagccagggggcgactcagatcccagccagtggacttagcccctgtttgctcctccgataactggggtgaccttggttaatattcaccagcagcctcccccgttgcccctctggatccactgcttaaatacggacgaggacagggccctgtctcctcagcttcaggcaccaccactgacctgggacagtgaatccctcgaggggcgcgccgccaccatgcaccagcgtcacccccgggcaagatgccctcccctctgtgtggccggaatccttgcctgtggctttctcctgggctgctggggaccctcccatttccagcagagttgtcttcaggctttggagccacaggccgtgtcttcttacttgagccctggtgctcccttaaaaggccgccctccttcccctggcttccagaggcagaggcagaggcagaggcgggctgcaggcggcatcctacacctggagctgctggtggccgtgggccccgatgtcttccaggctcaccaggaggacacagagcgctatgtgctcaccaacctcaacatcggggcagaactgcttcgggacccgtccctgggggctcagtttcgggtgcacctggtgaagatggtcattctgacagagcctgagggtgctccaaatatcacagccaacctcacctcgtccctgctgagcgtctgtgggtggagccagaccatcaaccctgaggacgacacagatcctggccatgctgacctggtcctctatatcactaggtttgacctggagttgcctgatggtaaccggcaggtgcggggcgtcacccagctgggcggtgcctgctccccaacctggagctgcctcattaccgaggacactggcttcgacctgggagtcaccattgcccatgagattgggcacagcttcggcctggagcacgacggagcgcccggcagcggctgcggccccagcggacacgtgatggcttcggacggagctgctcctagagctggcctcgcttggtccccctgcagcagacggcagctgctgagcctgctcagcgcaggacgggcgcgctgcgtgtgggacccgccgcggcctcaacccgggtccgcggggcacccgccggatgcgcagcctggcctctactacagcgccaacgagcagtgccgcgtggccttcggccccaaggctgtcgcctgcaccttcgccagggagcacctggatatgtgccaggccctctcctgccacacagacccgctggaccaaagcagctgcagccgcctcctcgttcctctcctggatgggacagaatgtggcgtggagaagtggtgctccaagggtcgctgccgctccctggtggagctgacccccatagcagcagtgcatgggcgctggtctagctggggtccccgaagtccttgctcccgctcctgcggaggaggtgtggtcaccaggaggcggcagtgcaacaaccccagacctgcctttggggggcgtgcatgtgttggtgctgacctccaggccgagatgtgcaacactcaggcctgcgagaagacccagctggagttcatgtcgcaacagtgcgccaggaccgacggccagccgctgcgctcctcccctggcggcgcctccttctaccactggggtgctgctgtaccacacagccaaggggatgctctgtgcagacacatgtgccgggccattggcgagagcttcatcatgaagcgtggagacagcttcctcgatgggacccggtgtatgccaagtggcccccgggaggacgggaccctgagcctgtgtgtgtcgggcagctgcaggacatttggctgtgatggtaggatggactcccagcaggtatgggacaggtgccaggtgtgtggtggggacaacagcacgtgcagcccacggaagggctctttcacagctggcagagcgagagaatatgtcacgtttctgacagttacccccaacctgaccagtgtctacattgccaaccacaggcctctcttcacacacttggcggtgaggatcggagggcgctatgtcgtggctgggaagatgagcatctcccctaacaccacctacccctccctcctggaggatggtcgtgtcgagtacagagtggccctcaccgaggaccggctgccccgcctggaggagatccgcatctggggacccctccaggaagatgctgacatccaggtttacaggcggtatggcgaggagtatggcaacctcacccgcccagacatcaccttcacctacttccagcctaagccacggcaggcctgggtgtgggccgctgtgcgtgggccctgctcggtgagctgtggggcagggctgcgctgggtaaactacagctgcctggaccaggccaggaaggagttggtggagactgtccagtgccaagggagccagcagccaccagcgtggccagaggcctgcgtgctcgaaccctgccctccctactggaaagtcatgtcccttggcccatgttcggccagctgtggccttggcactgctagacgctcggtggcctgtgtgcagctcgaccaaggccaggacgtggaggtggacgaggcggcctgtgcggcgctggtgcggcccgaggccagtgtcccctgtctcattgccgactgcacctaccgctggcatgttggcacctggatggagtgctctgtttcctgtggggatggcatccagcgccggcgtgacacctgcctcggaccccaggcccaggcgcctgtgccagctgatttctgccagcacttgcccaagccggtgactgtgcgtggctgctgggctgggccctgtgtgggacagggtacgcccagcctggtgccccacgaagaagccgctgctccaggacggaccacagccacccctgctggtgcctccctggagtggtcccaggcccggggcctgctcttctccccggctccccagcctcggcggctcctgcccgggccccaggaaaactcagtgcagtccagtgcctgtggcaggcagcaccttgagccaacaggaaccattgacatgcgaggcccagggcaggcagactgtgcagtggccattgggcggcccctcggggaggtggtgaccctccgcgtccttgagagttctctcaactgcagtgcgggggacatgttgctgctttggggccggctcacctggaggaagatgtgcaggaagctgttggacatgactttcagctccaagaccaacacgctggtggtgaggcagcgctgcgggcggccaggaggtggggtgctgctgcggtatgggagccagcttgctcctgaaaccttctacagagaatgtgacatgcagctctttgggccctggggtgaaatcgtgagcccctcgctgagtccagccacgagtaatgcagggggctgccggctcttcattaatgtggctccgcacgcacggattgccatccatgccctggccaccaacatgggcgctgggaccgagggagccaatgccagctacatcttgatccgggacacccacagcttgaggaccacagcgtttcatgggcagcaggtgctctactgggagtcagagagcagccaggctgagatggagttcagcgagggcttcctgaaggctcaggccagcctgcggggccagtattggaccctccaatcatgggtaccggagatgcaggaccctcagtcctggaagggaaaggaaggaacctgataagcggccgcaatcaaagcttaatcaacctctggattacaaaatttgtgaaagattgactggtattcttaactatgttgctccttttacgctatgtggatacgctgctttaatgcctttgtatcatgctattgcttcccgtatggctttcattttctcctccttgtataaatcctggttagttcttgccacggcggaactcatcgccgcctgccttgcccgctgctggacaggggctcggctgttgggcactgacaattccgtggtgttgagctcaataaaagatctttattttcattagatctgtgtgttggttttttgtgtggtcgaccggaccgagcggccgcggcgatctctaggaacccctagtgatggagttggccactccctctctgcgcgctcgctcgctcactgaggccgggcgaccaaaggtcgcccgacgcccgggctttgcccgggcggcctcagtgagcgagcgagcgcgcagctgcctgca

SEQ ID NO: 26 - DNA, 4565 bp, synthetic construct
  source 1..4565: mol_type = other DNA
tgcaggcagctgcgcgctcgctcgctcactgaggccgcccgggcaaagcccgggcgtcgggcgacctttggtcgcccggcctcagtgagcgagcgagcgcgcagagagggagtggccaactccatcactaggggttcctgatgcggctgcacgcgtgtgtttgctgcttgcaatgtttgcccattttagggtggacacaggacgctgtggtttctgagccagggggcgactcagatcccagccagtggacttagcccctgtttgctcctccgataactggggtgaccttggttaatattcaccagcagcctcccccgttgcccctctggatccactgcttaaatacggacgaggacagggccctgtctcctcagcttcaggcaccaccactgacctgggacagtgaatccggagtcgctgcgcgctgccttcgccccgtgccccgctccgccgccgcctcgcgccgcccgccccggctctgactgaccgcgttactcccacaggtgagcgggcgggacggcccttctccttcgggctgtaattagcgcttggtttaatgacggcttgtttcttttctgtggctgcgtgaaagccttgaggggctccgggagggccctttgtgcggggggagcggctcggggctgtccgcggggggacggctgccttcgggggggacggggcagggcggggttcggcttctggcgtgtgaccggcggctctagagcctctgctaaccatgttcatgccttcttctttttcctacagctcctgggcaacgtgctggttattgtgctgtctcatcattttggcaaagaattggatctcgaggggcgcgccgccaccatgcaccagcgtcacccccgggcaagatgccctcccctctgtgtggccggaatccttgcctgtggctttctcctgggctgctggggaccctcccatttccagcagagttgtcttcaggctttggagccacaggccgtgtcttcttacttgagccctggtgctcccttaaaaggccgccctccttcccctggcttccagaggcagaggcagaggcagaggcgggctgcaggcggcatcctacacctggagctgctggtggccgtgggccccgatgtcttccaggctcaccaggaggacacagagcgctatgtgctcaccaacctcaacatcggggcagaactgcttcgggacccgtccctgggggctcagtttcgggtgcacctggtgaagatggtcattctgacagagcctgagggtgctccaaatatcacagccaacctcacctcgtccctgctgagcgtctgtgggtggagccagaccatcaaccctgaggacgacacagatcctggccatgctgacctggtcctctatatcactaggtttgacctggagttgcctgatggtaaccggcaggtgcggggcgtcacccagctgggcggtgcctgctccccaacctggagctgcctcattaccgaggacactggcttcgacctgggagtcaccattgcccatgagattgggcacagcttcggcctggagcacgacggagcgcccggcagcggctgcggccccagcggacacgtgatggcttcggacggagctgctcctagagctggcctcgcttggtccccctgcagcagacggcagctgctgagcctgctcagcgcaggacgggcgcgctgcgtgtgggacccgccgcggcctcaacccgggtccgcggggcacccgccggatgcgcagcctggcctctactacagcgccaacgagcagtgccgcgtggccttcggccccaaggctgtcgcctgcaccttcgccagggagcacctggatatgtgccaggccctctcctgccacacagacccgctggaccaaagcagctgcagccgcctcctcgttcctctcctggatgggacagaatgtggcgtggagaagtggtgctccaagggtcgctgccgctccctggtggagctgacccccatagcagcagtgcatgggcgctggtctagctggggtccccgaagtccttgctcccgctcctgcggaggaggtgtggtcaccaggaggcggcagtgcaacaaccccagacctgcctttggggggcgtgcatgtgttggtgctgacctccaggccgagatgtgcaacactcaggcctgcgagaagacccagctggagttcatgtcgcaacagtgcgccaggaccgacggccagccgctgcgctcctcccctggcggcgcctccttctaccactggggtgctgctgtaccacacagccaaggggatgctctgtgcagacacatgtgccgggccattggcgagagcttcatcatgaagcgtggagacagcttcctcgatgggacccggtgtatgccaagtggcccccgggaggacgggaccctgagcctgtgtgtgtcgggcagctgcaggacatttggctgtgatggtaggatggactcccagcaggtatgggacaggtgccaggtgtgtggtggggacaacagcacgtgcagcccacggaagggctctttcacagctggcagagcgagagaatatgtcacgtttctgacagttacccccaacctgaccagtgtctacattgccaaccacaggcctctcttcacacacttggcggtgaggatcggagggcgctatgtcgtggctgggaagatgagcatctcccctaacaccacctacccctccctcctggaggatggtcgtgtcgagtacagagtggccctcaccgaggaccggctgccccgcctggaggagatccgcatctggggacccctccaggaagatgctgacatccaggtttacaggcggtatggcgaggagtatggcaacctcacccgcccagacatcaccttcacctacttccagcctaagccacggcaggcctgggtgtgggccgctgtgcgtgggccctgctcggtgagctgtggggcagggctgcgctgggtaaactacagctgcctggaccaggccaggaaggagttggtggagactgtccagtgccaagggagccagcagccaccagcgtggccagaggcctgcgtgctcgaaccctgccctccctactggaaagtcatgtcccttggcccatgttcggccagctgtggccttggcactgctagacgctcggtggcctgtgtgcagctcgaccaaggccaggacgtggaggtggacgaggcggcctgtgcggcgctggtgcggcccgaggccagtgtcccctgtctcattgccgactgcacctaccgctggcatgttggcacctggatggagtgctctgtttcctgtggggatggcatccagcgccggcgtgacacctgcctcggaccccaggcccaggcgcctgtgccagctgatttctgccagcacttgcccaagccggtgactgtgcgtggctgctgggctgggccctgtgtgggacagggtacgcccagcctggtgccccacgaagaagccgctgctccaggacggaccacagccacccctgctggtgcctccctggagtggtcccaggcccggggcctgctcttctccccggctccccagcctcggcggctcctgcccgggccccaggaaaactcagtgcagtccagtgcctgtggcaggcagcaccttgagccaacaggaaccattgacatgcgaggcccagggcaggcagactgtgcagtggccattgggcggcccctcggggaggtggtgaccctccgcgtccttgagagttctctcaactgcagtgcgggggacatgttgctgctttggggccggctcacctggaggaagatgtgcaggaagctgttggacatgactttcagctccaagaccaacacgctggtggtgaggcagcgctgcgggcggccaggaggtggggtgctgctgcggtatgggagccagcttgctcctgaaaccttctacagagaatgtgacatgcagctctttgggccctggggtgaaatcgtgagcccctcgctgagtccagccacgagtaatgcagggggctgccggctcttcattaatgtggctccgcacgcacggattgccatccatgccctggccaccaacatgggcgctgggaccgagggagccaatgccagctacatcttgatccgggacacccacagcttgaggaccacagcgtttcatgggcagcaggtgctctactgggagtcagagagcagccaggctgagatggagttcagcgagggcttcctgaaggctcaggccagcctgcggggccagtattggaccctccaatcatgggtaccggagatgcaggaccctcagtcctggaagggaaaggaaggaacctgataagcggccgcaatcaaagcttgagctcaataaaagatctttattttcattagatctgtgtgttggttttttgtgtggtcgaccggaccgagcggccgcggcgatctctaggaacccctagtgatggagttggccactccctctctgcgcgctcgctcgctcactgaggccgggcgaccaaaggtcgcccgacgcccgggctttgcccgggcggcctcagtgagcgagcgagcgcgcagctgcctgca

SEQ ID NO: 27 - DNA, 4813 bp, synthetic construct
  source 1..4813: mol_type = other DNA
tgcaggcagctgcgcgctcgctcgctcactgaggccgcccgggcaaagcccgggcgtcgggcgacctttggtcgcccggcctcagtgagcgagcgagcgcgcagagagggagtggccaactccatcactaggggttcctgatgcggctgcacgcgtgtgtttgctgcttgcaatgtttgcccattttagggtggacacaggacgctgtggtttctgagccagggggcgactcagatcccagccagtggacttagcccctgtttgctcctccgataactggggtgaccttggttaatattcaccagcagcctcccccgttgcccctctggatccactgcttaaatacggacgaggacagggccctgtctcctcagcttcaggcaccaccactgacctgggacagtgaatccggagtcgctgcgcgctgccttcgccccgtgccccgctccgccgccgcctcgcgccgcccgccccggctctgactgaccgcgttactcccacaggtgagcgggcgggacggcccttctccttcgggctgtaattagcgcttggtttaatgacggcttgtttcttttctgtggctgcgtgaaagccttgaggggctccgggagggccctttgtgcggggggagcggctcggggctgtccgcggggggacggctgccttcgggggggacggggcagggcggggttcggcttctggcgtgtgaccggcggctctagagcctctgctaaccatgttcatgccttcttctttttcctacagctcctgggcaacgtgctggttattgtgctgtctcatcattttggcaaagaattggatctcgaggggcgcgccgccaccatgcaccagcgtcacccccgggcaagatgccctcccctctgtgtggccggaatccttgcctgtggctttctcctgggctgctggggaccctcccatttccagcagagttgtcttcaggctttggagccacaggccgtgtcttcttacttgagccctggtgctcccttaaaaggccgccctccttcccctggcttccagaggcagaggcagaggcagaggcgggctgcaggcggcatcctacacctggagctgctggtggccgtgggccccgatgtcttccaggctcaccaggaggacacagagcgctatgtgctcaccaacctcaacatcggggcagaactgcttcgggacccgtccctgggggctcagtttcgggtgcacctggtgaagatggtcattctgacagagcctgagggtgctccaaatatcacagccaacctcacctcgtccctgctgagcgtctgtgggtggagccagaccatcaaccctgaggacgacacagatcctggccatgctgacctggtcctctatatcactaggtttgacctggagttgcctgatggtaaccggcaggtgcggggcgtcacccagctgggcggtgcctgctccccaacctggagctgcctcattaccgaggacactggcttcgacctgggagtcaccattgcccatgagattgggcacagcttcggcctggagcacgacggagcgcccggcagcggctgcggccccagcggacacgtgatggcttcggacggagctgctcctagagctggcctcgcttggtccccctgcagcagacggcagctgctgagcctgctcagcgcaggacgggcgcgctgcgtgtgggacccgccgcggcctcaacccgggtccgcggggcacccgccggatgcgcagcctggcctctactacagcgccaacgagcagtgccgcgtggccttcggccccaaggctgtcgcctgcaccttcgccagggagcacctggatatgtgccaggccctctcctgccacacagacccgctggaccaaagcagctgcagccgcctcctcgttcctctcctggatgggacagaatgtggcgtggagaagtggtgctccaagggtcgctgccgctccctggtggagctgacccccatagcagcagtgcatgggcgctggtctagctggggtccccgaagtccttgctcccgctcctgcggaggaggtgtggtcaccaggaggcggcagtgcaacaaccccagacctgcctttggggggcgtgcatgtgttggtgctgacctccaggccgagatgtgcaacactcaggcctgcgagaagacccagctggagttcatgtcgcaacagtgcgccaggaccgacggccagccgctgcgctcctcccctggcggcgcctccttctaccactggggtgctgctgtaccacacagccaaggggatgctctgtgcagacacatgtgccgggccattggcgagagcttcatcatgaagcgtggagacagcttcctcgatgggacccggtgtatgccaagtggcccccgggaggacgggaccctgagcctgtgtgtgtcgggcagctgcaggacatttggctgtgatggtaggatggactcccagcaggtatgggacaggtgccaggtgtgtggtggggacaacagcacgtgcagcccacggaagggctctttcacagctggcagagcgagagaatatgtcacgtttctgacagttacccccaacctgaccagtgtctacattgccaaccacaggcctctcttcacacacttggcggtgaggatcggagggcgctatgtcgtggctgggaagatgagcatctcccctaacaccacctacccctccctcctggaggatggtcgtgtcgagtacagagtggccctcaccgaggaccggctgccccgcctggaggagatccgcatctggggacccctccaggaagatgctgacatccaggtttacaggcggtatggcgaggagtatggcaacctcacccgcccagacatcaccttcacctacttccagcctaagccacggcaggcctgggtgtgggccgctgtgcgtgggccctgctcggtgagctgtggggcagggctgcgctgggtaaactacagctgcctggaccaggccaggaaggagttggtggagactgtccagtgccaagggagccagcagccaccagcgtggccagaggcctgcgtgctcgaaccctgccctccctactggaaagtcatgtcccttggcccatgttcggccagctgtggccttggcactgctagacgctcggtggcctgtgtgcagctcgaccaaggccaggacgtggaggtggacgaggcggcctgtgcggcgctggtgcggcccgaggccagtgtcccctgtctcattgccgactgcacctaccgctggcatgttggcacctggatggagtgctctgtttcctgtggggatggcatccagcgccggcgtgacacctgcctcggaccccaggcccaggcgcctgtgccagctgatttctgccagcacttgcccaagccggtgactgtgcgtggctgctgggctgggccctgtgtgggacagggtacgcccagcctggtgccccacgaagaagccgctgctccaggacggaccacagccacccctgctggtgcctccctggagtggtcccaggcccggggcctgctcttctccccggctccccagcctcggcggctcctgcccgggccccaggaaaactcagtgcagtccagtgcctgtggcaggcagcaccttgagccaacaggaaccattgacatgcgaggcccagggcaggcagactgtgcagtggccattgggcggcccctcggggaggtggtgaccctccgcgtccttgagagttctctcaactgcagtgcgggggacatgttgctgctttggggccggctcacctggaggaagatgtgcaggaagctgttggacatgactttcagctccaagaccaacacgctggtggtgaggcagcgctgcgggcggccaggaggtggggtgctgctgcggtatgggagccagcttgctcctgaaaccttctacagagaatgtgacatgcagctctttgggccctggggtgaaatcgtgagcccctcgctgagtccagccacgagtaatgcagggggctgccggctcttcattaatgtggctccgcacgcacggattgccatccatgccctggccaccaacatgggcgctgggaccgagggagccaatgccagctacatcttgatccgggacacccacagcttgaggaccacagcgtttcatgggcagcaggtgctctactgggagtcagagagcagccaggctgagatggagttcagcgagggcttcctgaaggctcaggccagcctgcggggccagtattggaccctccaatcatgggtaccggagatgcaggaccctcagtcctggaagggaaaggaaggaacctgataagcggccgcaatcaaagcttaatcaacctctggattacaaaatttgtgaaagattgactggtattcttaactatgttgctccttttacgctatgtggatacgctgctttaatgcctttgtatcatgctattgcttcccgtatggctttcattttctcctccttgtataaatcctggttagttcttgccacggcggaactcatcgccgcctgccttgcccgctgctggacaggggctcggctgttgggcactgacaattccgtggtgttgagctcaataaaagatctttattttcattagatctgtgtgttggttttttgtgtggtcgaccggaccgagcggccgcggcgatctctaggaacccctagtgatggagttggccactccctctctgcgcgctcgctcgctcactgaggccgggcgaccaaaggtcgcccgacgcccgggctttgcccgggcggcctcagtgagcgagcgagcgcgcagctgcctgca

SEQ ID NO: 28 - DNA, 17 bp, synthetic construct
  source 1..17: mol_type = other DNA
tggaggagatccgcatc

SEQ ID NO: 29 - DNA, 21 bp, synthetic construct
  source 1..21: mol_type = other DNA
cgcctgtaaacctggatgtca

SEQ ID NO: 30 - DNA, 15 bp, synthetic construct
  source 1..15: mol_type = other DNA
acccctccaggaaga

SEQ ID NO: 31 - DNA, 2611 bp, synthetic construct
  source 1..2611: mol_type = other DNA
cctgcaggcagctgcgcgctcgctcgctcactgaggccgcccgggcgtcgggcgacctttggtcgcccggcctcagtgagcgagcgagcgcgcagagagggagtggccaactccatcactaggggttcctgcggccgcacgcgtggttaatcattaagtcgttaatttttgtggcccttgcgatgtttgctctggttaataatctcaggacaaacagaggttaataattttccagatctctctgagcaatagtataaaaggccagcagcagcctgaccacatctcatcctccctcgaggggcgcgccgccaccatgcaccagcgtcacccccgggcaagatgccctcccctctgtgtggccggaatccttgcctgtggctttctcctgggctgctggggaccctcccatttccagcagagttgtcttcaggctttggagccacaggccgtgtcttcttacttgagccctggtgctcccttaaaaggccgccctccttcccctggcttccagaggcagaggcagaggcagaggcgggctgcaggcggcatcctacacctggagctgctggtggccgtgggccccgatgtcttccaggctcaccaggaggacacagagcgctatgtgctcaccaacctcaacatcggggcagaactgcttcgggacccgtccctgggggctcagtttcgggtgcacctggtgaagatggtcattctgacagagcctgagggtgctccaaatatcacagccaacctcacctcgtccctgctgagcgtctgtgggtggagccagaccatcaaccctgaggacgacacagatcctggccatgctgacctggtcctctatatcactaggtttgacctggagttgcctgatggtaaccggcaggtgcggggcgtcacccagctgggcggtgcctgctccccaacctggagctgcctcattaccgaggacactggcttcgacctgggagtcaccattgcccatgagattgggcacagcttcggcctggagcacgacggagcgcccggcagcggctgcggccccagcggacacgtgatggcttcggacggagctgctcctagagctggcctcgcttggtccccctgcagcagacggcagctgctgagcctgctcagcgcaggacgggcgcgctgcgtgtgggacccgccgcggcctcaacccgggtccgcggggcacccgccggatgcgcagcctggcctctactacagcgccaacgagcagtgccgcgtggccttcggccccaaggctgtcgcctgcaccttcgccagggagcacctggatatgtgccaggccctctcctgccacacagacccgctggaccaaagcagctgcagccgcctcctcgttcctctcctggatgggacagaatgtggcgtggagaagtggtgctccaagggtcgctgccgctccctggtggagctgacccccatagcagcagtgcatgggcgctggtctagctggggtccccgaagtccttgctcccgctcctgcggaggaggtgtggtcaccaggaggcggcagtgcaacaaccccagacctgcctttggggggcgtgcatgtgttggtgctgacctccaggccgagatgtgcaacactcaggcctgcgagaagacccagctggagttcatgtcgcaacagtgcgccaggaccgacggccagccgctgcgctcctcccctggcggcgcctccttctaccactggggtgctgctgtaccacacagccaaggggatgctctgtgcagacacatgtgccgggccattggcgagagcttcatcatgaagcgtggagacagcttcctcgatgggacccggtgtatgccaagtggcccccgggaggacgggaccctgagcctgtgtgtgtcgggcagctgcaggacatttggctgtgatggtaggatggactcccagcaggtatgggacaggtgccaggtgtgtggtggggacaacagcacgtgcagcccacggaagggctctttcacagctggcagagcgagagaatatgtcacgtttctgacagttacccccaacctgaccagtgtctacattgccaaccacaggcctctcttcacacacttggcggtgaggatcggagggcgctatgtcgtggctgggaagatgagcatctcccctaacaccacctacccctccctcctggaggatggtcgtgtcgagtacagagtggccctcaccgaggaccggctgccccgcctggaggagatccgcatctggggacccctccaggaagatgctgacatccaggtttacaggcggtatggcgaggagtatggcaacctcacccgcccagacatcaccttcacctacttccagcctaagccacggcaggcctgataagcggccgcaatcaaagcttgagctcaataaaagatctttattttcattagatctgtgtgttggttttttgtgtggtcgaccggaccgagcggccgcaggaacccctagtgatggagttggccactccctctctgcgcgctcgctcgctcactgaggccgggcgaccaaaggtcgcccgacgcccgggctttgcccgggcggcctcagtgagcgagcgagcgcgcagctgcctgcagg

SEQ ID NO: 32 - DNA, 304 bp, synthetic construct
  source 1..304: mol_type = other DNA
cgttacataacttacggtaaatggcccgcctggctgaccgcccaacgacccccgcccattgacgtcaataatgacgtatgttcccatagtaacgtcaatagggactttccattgacgtcaatgggtggagtatttacggtaaactgcccacttggcagtacatcaagtgtatcatatgccaagtacgccccctattgacgtcaatgacggtaaatggcccgcctggcattatgcccagtacatgaccttatgggactttcctacttggcagtacatctacgtattagtcatcgctattaccatg

SEQ ID NO: 33 - DNA, 203 bp, synthetic construct
  source 1..203: mol_type = other DNA
gtgatgcggttttggcagtacatcaatgggcgtggatagcggtttgactcacggggatttccaagtctccaccccattgacgtcaatgggagtttgttttgcaccaaaatcaacgggactttccaaaatgtcgtaacaactccgccccattgacgcaaatgggcggtaggcgtgtacggtgggaggtctatataagcagagct

SEQ ID NO: 34 - DNA, 477 bp, synthetic construct
  source 1..477: mol_type = other DNA
gggtggcatccctgtgacccctccccagtgcctctcctggccctggaagttgccactccagtgcccaccagccttgtcctaataaaattaagttgcatcattttgtctgactaggtgtccttctataatattatggggtggaggggggtggtatggagcaaggggcaagttgggaagacaacctgtagggcctgcggggtctattgggaaccaagctggagtgcagtggcacaatcttggctcactgcaatctccgcctcctgggttcaagcgattctcctgcctcagcctcccgagttgttgggattccaggcatgcatgaccaggctcagctaatttttgtttttttggtagagacggggtttcaccatattggccaggctggtctccaactcctaatctcaggtgatctacccaccttggcctcccaaattgctgggattacaggcgtgaaccactgctcccttccctgtcctt

SEQ ID NO: 35 - DNA, 49 bp, synthetic construct
  source 1..49: mol_type = other DNA
aataaaagatctttattttcattagatctgtgtgttggttttttgtgtg

SEQ ID NO: 36 - DNA, 252 bp, synthetic construct
  source 1..252: mol_type = other DNA
tgtttgctgcttgcaatgtttgcccattttagggtggacacaggacgctgtggtttctgagccagggggcgactcagatcccagccagtggacttagcccctgtttgctcctccgataactggggtgaccttggttaatattcaccagcagcctcccccgttgcccctctggatccactgcttaaatacggacgaggacagggccctgtctcctcagcttcaggcaccaccactgacctgggacagtgaatc

SEQ ID NO: 37 - DNA, 146 bp, synthetic construct
  source 1..146: mol_type = other DNA
gttaatcattaagtcgttaatttttgtggcccttgcgatgtttgctctggttaataatctcaggacaaacagaggttaataattttccagatctctctgagcaatagtataaaaggccagcagcagcctgaccacatctcatcctc

SEQ ID NO: 38 - DNA, 130 bp, synthetic construct
  source 1..130: mol_type = other DNA
cctgcaggcagctgcgcgctcgctcgctcactgaggccgcccgggcgtcgggcgacctttggtcgcccggcctcagtgagcgagcgagcgcgcagagagggagtggccaactccatcactaggggttcct

SEQ ID NO: 39 - DNA, 141 bp, synthetic construct
  source 1..141: mol_type = other DNA
aggaacccctagtgatggagttggccactccctctctgcgcgctcgctcgctcactgaggccgggcgaccaaaggtcgcccgacgcccgggctttgcccgggcggcctcagtgagcgagcgagcgcgcagctgcctgcagg

SEQ ID NO: 40 - DNA, 493 bp, synthetic construct
  source 1..493: mol_type = other DNA
cgaatcccggccgggaacggtgcattggaacgcggattccccgtgccaagagtgacgtaagtaccgcctatagagtctataggcccacaaaaaatgctttcttcttttaatatacttttttgtttatcttatttctaatactttccctaatctctttctttcagggcaataatgatacaatgtatcatgcctctttgcaccattctaaagaataacagtgataatttctgggttaaggcaatagcaatatttctgcatataaatatttctgcatataaattgtaactgatgtaagaggtttcatattgctaatagcagctacaatccagctaccattctgcttttattttatggttgggataaggctggattattctgagtccaagctaggcccttttgctaatcatgttcatacctcttatcttcctcccacagctcctgggcaacgtgctggtctgtgtgctggcccatcactttggcaaagaattgggat

SEQ ID NO: 41 - DNA, 3897 bp, synthetic construct
  source 1..3897: mol_type = other DNA
atgcaccagcgtcacccccgggcaagatgccctcccctctgtgtggccggaatccttgcctgtggctttctcctgggctgctggggaccctcccatttccagcagagttgtcttcaggctttggagccacaggccgtgtcttcttacttgagccctggtgctcccttaaaaggccgccctccttcccctggcttccagaggcagaggcagaggcagaggcgggctgcaggcggcatcctacacctggagctgctggtggccgtgggccccgatgtcttccaggctcaccaggaggacacagagcgctatgtgctcaccaacctcaacatcggggcagaactgcttcgggacccgtccctgggggctcagtttcgggtgcacctggtgaagatggtcattctgacagagcctgagggtgctccaaatatcacagccaacctcacctcgtccctgctgagcgtctgtgggtggagccagaccatcaaccctgaggacgacacagatcctggccatgctgacctggtcctctatatcactaggtttgacctggagttgcctgatggtaaccggcaggtgcggggcgtcacccagctgggcggtgcctgctccccaacctggagctgcctcattaccgaggacactggcttcgacctgggagtcaccattgcccatgagattgggcacagcttcggcctggagcacgacggagcgcccggcagcggctgcggccccagcggacacgtgatggcttcggacggagctgctcctagagctggcctcgcttggtccccctgcagcagacggcagctgctgagcctgctcagcgcaggacgggcgcgctgcgtgtgggacccgccgcggcctcaacccgggtccgcggggcacccgccggatgcgcagcctggcctctactacagcgccaacgagcagtgccgcgtggccttcggccccaaggctgtcgcctgcaccttcgccagggagcacctggatatgtgccaggccctctcctgccacacagacccgctggaccaaagcagctgcagccgcctcctcgttcctctcctggatgggacagaatgtggcgtggagaagtggtgctccaagggtcgctgccgctccctggtggagctgacccccatagcagcagtgcatgggcgctggtctagctggggtccccgaagtccttgctcccgctcctgcggaggaggtgtggtcaccaggaggcggcagtgcaacaaccccagacctgcctttggggggcgtgcatgtgttggtgctgacctccaggccgagatgtgcaacactcaggcctgcgagaagacccagctggagttcatgtcgcaacagtgcgccaggaccgacggccagccgctgcgctcctcccctggcggcgcctccttctaccactggggtgctgctgtaccacacagccaaggggatgctctgtgcagacacatgtgccgggccattggcgagagcttcatcatgaagcgtggagacagcttcctcgatgggacccggtgtatgccaagtggcccccgggaggacgggaccctgagcctgtgtgtgtcgggcagctgcaggacatttggctgtgatggtaggatggactcccagcaggtatgggacaggtgccaggtgtgtggtggggacaacagcacgtgcagcccacggaagggctctttcacagctggcagagcgagagaatatgtcacgtttctgacagttacccccaacctgaccagtgtctacattgccaaccacaggcctctcttcacacacttggcggtgaggatcggagggcgctatgtcgtggctgggaagatgagcatctcccctaacaccacctacccctccctcctggaggatggtcgtgtcgagtacagagtggccctcaccgaggaccggctgccccgcctggaggagatccgcatctggggacccctccaggaagatgctgacatccaggtttacaggcggtatggcgaggagtatggcaacctcacccgcccagacatcaccttcacctacttccagcctaagccacggcaggcctgggtgtgggccgctgtgcgtgggccctgctcggtgagctgtggggcagggctgcgctgggtaaactacagctgcctggaccaggccaggaaggagttggtggagactgtccagtgccaagggagccagcagccaccagcgtggccagaggcctgcgtgctcgaaccctgccctccctactgggcggtgggagacttcggcccatgcagcgcctcctgtgggggtggcctgcgggagcggccagtgcgctgcgtggaggcccagggcagcctcctgaagacattgcccccagcccggtgcagagcaggggcccagcagccagctgtggcgctggaaacctgcaacccccagccctgccctgccaggtgggaggtgtcagagcccagctcatgcacatcagctggtggagcaggcctggccttggagaacgagacctgtgtgccaggggcagatggcctggaggctccagtgactgaggggcctggctccgtagatgagaagctgcctgcccctgagccctgtgtcgggatgtcatgtcctccaggctggggccatctggatgccacctctgcaggggagaaggctccctccccttggggcagcatcaggacgggggctcaagctgcacacgtgtggacccctgcggcagggtcgtgctccgtctcctgcgggcgaggtctgatggagctgcgtttcctgtgcatggactctgccctcagggtgcctgtccaggaagagctgtgtggcctggcaagcaagcctgggagccggcgggaggtctgccaggctgtcccgtgccctgctcggtggcagtacaagctggcggcctgcagcgtgagctgtgggagaggggtcgtgcggagaatcctgtattgtgcccgggctcatggggaggacgatggtgaggagatcctgttggacacccagtgccaggggctgcctcgcccggaaccccaggaggcctgcagcctggagccctgcccacctaggtggaaagtcatgtcccttggcccatgttcggccagctgtggccttggcactgctagacgctcggtggcctgtgtgcagctcgaccaaggccaggacgtggaggtggacgaggcggcctgtgcggcgctggtgcggcccgaggccagtgtcccctgtctcattgccgactgcacctaccgctggcatgttggcacctggatggagtgctctgtttcctgtggggatggcatccagcgccggcgtgacacctgcctcggaccccaggcccaggcgcctgtgccagctgatttctgccagcacttgcccaagccggtgactgtgcgtggctgctgggctgggccctgtgtgggacagggtacgcccagcctggtgccccacgaagaagccgctgctccaggacggaccacagccacccctgctggtgcctccctggagtggtcccaggcccggggcctgctcttctccccggctccccagcctcggcggctcctgcccgggccccaggaaaactcagtgcagtccagtgcctgtggcaggcagcaccttgagccaacaggaaccattgacatgcgaggcccagggcaggcagactgtgcagtggccattgggcggcccctcggggaggtggtgaccctccgcgtccttgagagttctctcaactgcagtgcgggggacatgttgctgctttggggccggctcacctggaggaagatgtgcaggaagctgttggacatgactttcagctccaagaccaacacgctggtggtgaggcagcgctgcgggcggccaggaggtggggtgctgctgcggtatgggagccagcttgctcctgaaaccttctacagagaatga

SEQ ID NO: 42 - DNA, 3087 bp, synthetic construct
  source 1..3087: mol_type = other DNA
atgcaccagcgtcacccccgggcaagatgccctcccctctgtgtggccggaatccttgcctgtggctttctcctgggctgctggggaccctcccatttccagcagagttgtcttcaggctttggagccacaggccgtgtcttcttacttgagccctggtgctcccttaaaaggccgccctccttcccctggcttccagaggcagaggcagaggcagaggcgggctgcaggcggcatcctacacctggagctgctggtggccgtgggccccgatgtcttccaggctcaccaggaggacacagagcgctatgtgctcaccaacctcaacatcggggcagaactgcttcgggacccgtccctgggggctcagtttcgggtgcacctggtgaagatggtcattctgacagagcctgagggtgctccaaatatcacagccaacctcacctcgtccctgctgagcgtctgtgggtggagccagaccatcaaccctgaggacgacacagatcctggccatgctgacctggtcctctatatcactaggtttgacctggagttgcctgatggtaaccggcaggtgcggggcgtcacccagctgggcggtgcctgctccccaacctggagctgcctcattaccgaggacactggcttcgacctgggagtcaccattgcccatgagattgggcacagcttcggcctggagcacgacggagcgcccggcagcggctgcggccccagcggacacgtgatggcttcggacggagctgctcctagagctggcctcgcttggtccccctgcagcagacggcagctgctgagcctgctcagcgcaggacgggcgcgctgcgtgtgggacccgccgcggcctcaacccgggtccgcggggcacccgccggatgcgcagcctggcctctactacagcgccaacgagcagtgccgcgtggccttcggccccaaggctgtcgcctgcaccttcgccagggagcacctggatatgtgccaggccctctcctgccacacagacccgctggaccaaagcagctgcagccgcctcctcgttcctctcctggatgggacagaatgtggcgtggagaagtggtgctccaagggtcgctgccgctccctggtggagctgacccccatagcagcagtgcatgggcgctggtctagctggggtccccgaagtccttgctcccgctcctgcggaggaggtgtggtcaccaggaggcggcagtgcaacaaccccagacctgcctttggggggcgtgcatgtgttggtgctgacctccaggccgagatgtgcaacactcaggcctgcgagaagacccagctggagttcatgtcgcaacagtgcgccaggaccgacggccagccgctgcgctcctcccctggcggcgcctccttctaccactggggtgctgctgtaccacacagccaaggggatgctctgtgcagacacatgtgccgggccattggcgagagcttcatcatgaagcgtggagacagcttcctcgatgggacccggtgtatgccaagtggcccccgggaggacgggaccctgagcctgtgtgtgtcgggcagctgcaggacatttggctgtgatggtaggatggactcccagcaggtatgggacaggtgccaggtgtgtggtggggacaacagcacgtgcagcccacggaagggctctttcacagctggcagagcgagagaatatgtcacgtttctgacagttacccccaacctgaccagtgtctacattgccaaccacaggcctctcttcacacacttggcggtgaggatcggagggcgctatgtcgtggctgggaagatgagcatctcccctaacaccacctacccctccctcctggaggatggtcgtgtcgagtacagagtggccctcaccgaggaccggctgccccgcctggaggagatccgcatctggggacccctccaggaagatgctgacatccaggtttacaggcggtatggcgaggagtatggcaacctcacccgcccagacatcaccttcacctacttccagcctaagccacggcaggcctgggtgtgggccgctgtgcgtgggccctgctcggtgagctgtggggcagggctgcgctgggtaaactacagctgcctggaccaggccaggaaggagttggtggagactgtccagtgccaagggagccagcagccaccagcgtggccagaggcctgcgtgctcgaaccctgccctccctactggaaagtcatgtcccttggcccatgttcggccagctgtggccttggcactgctagacgctcggtggcctgtgtgcagctcgaccaaggccaggacgtggaggtggacgaggcggcctgtgcggcgctggtgcggcccgaggccagtgtcccctgtctcattgccgactgcacctaccgctggcatgttggcacctggatggagtgctctgtttcctgtggggatggcatccagcgccggcgtgacacctgcctcggaccccaggcccaggcgcctgtgccagctgatttctgccagcacttgcccaagccggtgactgtgcgtggctgctgggctgggccctgtgtgggacagggtacgcccagcctggtgccccacgaagaagccgctgctccaggacggaccacagccacccctgctggtgcctccctggagtggtcccaggcccggggcctgctcttctccccggctccccagcctcggcggctcctgcccgggccccaggaaaactcagtgcagtccagtgcctgtggcaggcagcaccttgagccaacaggaaccattgacatgcgaggcccagggcaggcagactgtgcagtggccattgggcggcccctcggggaggtggtgaccctccgcgtccttgagagttctctcaactgcagtgcgggggacatgttgctgctttggggccggctcacctggaggaagatgtgcaggaagctgttggacatgactttcagctccaagaccaacacgctggtggtgaggcagcgctgcgggcggccaggaggtggggtgctgctgcggtatgggagccagcttgctcctgaaaccttctacagagaatga